European Patent Application EP 4 270 006 A2, published November 1, 2023. Title: Detection and isolation of specific cells by binding of labelled molecules. Applicant: Immudex ApS. Application EP. The sequence listing filed with the application follows.

SEQUENCE LISTING (606 sequences)

SEQ ID NO: 1 - DNA, 69 bp, synthetic construct
  misc_feature 1..69: note = Barcode for CMV, Biotin-TEG at 5' end
  misc_feature 1..69: note = Barcode for CMV
  misc_feature 13..18: note = n: any of A, T, G, C independently
  source 1..69: mol_type = other DNA
gagatacgttgacctcgttgaannnnnntctatccattccatccagctcacttaagctcttggttgcat

SEQ ID NO: 2 - DNA, 69 bp, synthetic construct
  misc_feature 1..69: note = Barcode for HIV, Biotin-TEG at 5' end
  misc_feature 1..69: note = Barcode for HIV
  misc_feature 13..18: note = n: any of A, T, G, C independently
  source 1..69: mol_type = other DNA
gagatacgttgacctcgttgaannnnnntctataggtgtctactacctcacttaagctcttggttgcat

SEQ ID NO: 3 - DNA, 20 bp, synthetic construct
  misc_feature 1..20: note = Forward-01 primer
  primer_bind 1..20: note = Forward-01 primer
  source 1..20: mol_type = other DNA
gagatacgttgacctcgttg

SEQ ID NO: 4 - DNA, 20 bp, synthetic construct
  misc_feature 1..20: note = Reverse-01 primer
  primer_bind 1..20: note = Reverse-01 primer
  source 1..20: mol_type = other DNA
atgcaaccaagagcttaagt

SEQ ID NO: 5 - DNA, 69 bp, synthetic construct; identical to SEQ ID NO: 1
  misc_feature 1..69: note = TestOligo-01, biotin-TEG at 5' end
  misc_feature 1..69: note = TestOligo-01
  misc_feature 13..18: note = n: any of A, T, G, C independently
  source 1..69: mol_type = other DNA

SEQ ID NO: 6 - DNA, 69 bp, synthetic construct; identical to SEQ ID NO: 1
  misc_feature 1..69: note = TestOligo-02, biotin-TEG at 5' end followed by HEG (terminal modifications)
  misc_feature 1..69: note = TestOligo-02
  misc_feature 13..18: note = n: any of A, T, G, C independently
  source 1..69: mol_type = other DNA

SEQ ID NO: 7 - DNA, 69 bp, synthetic construct; identical to SEQ ID NO: 1
  misc_feature 1..69: note = TestOligo-03, biotin-TEG at 5' end followed by HEG (terminal modifications) and HEG at 3' end
  misc_feature 1..69: note = TestOligo-03
  misc_feature 13..18: note = n: any of A, T, G, C independently
  source 1..69: mol_type = other DNA

SEQ ID NO: 8 - DNA, 69 bp, synthetic construct
  misc_feature 1..69: note = TestOligo-04, biotin-TEG at 5' end followed by HEG (terminal modifications) and HEG at 3' end
  misc_feature 1..69: note = TestOligo-04
  misc_feature 13..18: note = n: any of A, T, G, C independently
  source 1..69: mol_type = other DNA
gagatacgttgacctcgttgaannnnnntcttgaactatgaatcgtctcacttaagctcttggttgcat

SEQ ID NO: 9 - DNA, 69 bp, synthetic construct; identical to SEQ ID NO: 2
  misc_feature 1..69: note = TestOligo-05, biotin-TEG at 5' end followed by HEG (terminal modifications) and HEG at 3' end
  misc_feature 1..69: note = TestOligo-05
  misc_feature 13..18: note = n: any of A, T, G, C
  source 1..69: mol_type = other DNA

SEQ ID NO: 10 - DNA, 69 bp, synthetic construct
  misc_feature 1..69: note = TestOligo-06, biotin-TEG at 5' end followed by HEG (terminal modifications) and HEG at 3' end
  misc_feature 1..69: note = TestOligo-06
  misc_feature 13..18: note = n: any of A, T, G, C independently
  source 1..69: mol_type = other DNA
gagatacgttgacctcgttgaannnnnntctttattggagagcacgctcacttaagctcttggttgcat

SEQ ID NO: 11 - DNA, 19 bp, synthetic construct
  misc_feature 1..19: note = LNA-3, 6FAM in 5', BHQ-1-plus in 3'
  misc_feature 1..19: note = LNA-3
  misc_feature 4..6: note = LNA modified RNA nucleotides
  misc_feature 9..10: note = LNA modified RNA nucleotides
  misc_feature 13..15: note = LNA modified RNA nucleotides
  source 1..19: mol_type = other DNA
tctatccattccatccagc

SEQ ID NO: 12 - DNA, 19 bp, synthetic construct
  misc_feature 1..19: note = LNA-4, 6FAM in 5'. BHQ-1-plus in 3'
  misc_feature 1..19: note = LNA-4
  misc_feature 4..6: note = LNA modified RNA nucleotides
  misc_feature 9..10: note = LNA modified RNA nucleotides
  misc_feature 13..15: note = LNA modified RNA nucleotides
  source 1..19: mol_type = other DNA
tcttgaactatgaatcgtc

SEQ ID NO: 13 - DNA, 19 bp, synthetic construct
  misc_feature 1..19: note = LNA-5, HEX in 5', BHQ-1-plus in 3'
  misc_feature 1..19: note = LNA-5
  misc_feature 4..6: note = LNA modified RNA nucleotides
  misc_feature 9..10: note = LNA modified RNA nucleotides
  misc_feature 13..15: note = LNA modified RNA nucleotides
  source 1..19: mol_type = other DNA
tctataggtgtctactacc

SEQ ID NO: 14 - DNA, 19 bp, synthetic construct
  misc_feature 1..19: note = LNA-6, cyanine 5 in 5'-end; bhq-2-plus in 3' end
  misc_feature 1..19: note = LNA-6
  misc_feature 4..6: note = LNA modified RNA nucleotides
  misc_feature 9..10: note = LNA modified RNA nucleotides
  misc_feature 13..15: note = LNA modified RNA nucleotides
  source 1..19: mol_type = other DNA
tctttattggagagcacgc

SEQ ID NO: 15 - protein, 9 aa, synthetic construct
  REGION 1..9: note = Negative control
  PEPTIDE 1..9: note = Dextramer 3, Negative (HLA-A*0201/ALIAPVHAV/Neg.Control).
ALIAPVHAV

SEQ ID NO: 16 - DNA, 58 bp, synthetic construct
  misc_feature 1..58: note = A-key 1OS-F1-1
  misc_feature 1..58: note = A-key 1OS-F1-1
  source 1..58: mol_type = other DNA
ccatctcatccctgcgtgtctccgactcaggaagatgattctataaactgtgcggtcc

SEQ ID NO: 17 - DNA, 58 bp, synthetic construct
  misc_feature 1..58: note = A-key 1OS-F1-2
  misc_feature 1..58: note = A-key 1OS-F1-2
  source 1..58: mol_type = other DNA
ccatctcatccctgcgtgtctccgactcagtcctgagattctataaactgtgcggtcc

SEQ ID NO: 18 - DNA, 58 bp, synthetic construct
  misc_feature 1..58: note = A-key 1OS-F1-3
  misc_feature 1..58: note = A-key 1OS-F1-3
  source 1..58: mol_type = other DNA
ccatctcatccctgcgtgtctccgactcagtgtggagattctataaactgtgcggtcc

SEQ ID NO: 19 - DNA, 58 bp, synthetic construct
  misc_feature 1..58: note = A-key 1OS-F1-4
  misc_feature 1..58: note = A-key 1OS-F1-4
  source 1..58: mol_type = other DNA
ccatctcatccctgcgtgtctccgactcagcatttagattctataaactgtgcggtcc

SEQ ID NO: 20 - DNA, 58 bp, synthetic construct
  misc_feature 1..58: note = A-key 1OS-F1-5
  misc_feature 1..58: note = A-key 1OS-F1-5
  source 1..58: mol_type = other DNA
ccatctcatccctgcgtgtctccgactcagttacccgattctataaactgtgcggtcc

SEQ ID NO: 21 - DNA, 58 bp, synthetic construct
  misc_feature 1..58: note = A-key 1OS-F1-6
  misc_feature 1..58: note = A-key 1OS-F1-6
  source 1..58: mol_type = other DNA
ccatctcatccctgcgtgtctccgactcagattctcgattctataaactgtgcggtcc

SEQ ID NO: 22 - DNA, 58 bp, synthetic construct
  misc_feature 1..58: note = A-key 1OS-F1-7
  misc_feature 1..58: note = A-key 1OS-F1-7
  source 1..58: mol_type = other DNA
ccatctcatccctgcgtgtctccgactcagagacccgattctataaactgtgcggtcc

SEQ ID NO: 23 - DNA, 58 bp, synthetic construct
  misc_feature 1..58: note = A-key 1OS-F1-8
  misc_feature 1..58: note = A-key 1OS-F1-8
  source 1..58: mol_type = other DNA
ccatctcatccctgcgtgtctccgactcagcgcatggattctataaactgtgcggtcc

SEQ ID NO: 24 - DNA, 58 bp, synthetic construct
  misc_feature 1..58: note = A-key 1OS-F1-9
  misc_feature 1..58: note = A-key 1OS-F1-9
  source 1..58: mol_type = other DNA
ccatctcatccctgcgtgtctccgactcagtcctcggattctataaactgtgcggtcc

SEQ ID NO: 25 - DNA, 58 bp, synthetic construct
  misc_feature 1..58: note = A-key 1OS-F1-10
  misc_feature 1..58: note = A-key 1OS-F1-10
  source 1..58: mol_type = other DNA
ccatctcatccctgcgtgtctccgactcagattcctgattctataaactgtgcggtcc

SEQ ID NO: 26 - DNA, 58 bp, synthetic construct
  misc_feature 1..58: note = A-key 1OS-F1-11
  misc_feature 1..58: note = A-key 1OS-F1-11
  source 1..58: mol_type = other DNA
ccatctcatccctgcgtgtctccgactcagcgtcgagattctataaactgtgcggtcc

SEQ ID NO: 27 - DNA, 58 bp, synthetic construct
  misc_feature 1..58: note = A-key 1OS-F1-12
  misc_feature 1..58: note = A-key 1OS-F1-12
  source 1..58: mol_type = other DNA
ccatctcatccctgcgtgtctccgactcaggccaatgattctataaactgtgcggtcc

SEQ ID NO: 28 - DNA, 58 bp, synthetic construct
  misc_feature 1..58: note = A-key 1OS-F1-13
  misc_feature 1..58: note = A-key 1OS-F1-13
  source 1..58: mol_type = other DNA
ccatctcatccctgcgtgtctccgactcagatacgggattctataaactgtgcggtcc

SEQ ID NO: 29 - DNA, 58 bp, synthetic construct
  misc_feature 1..58: note = A-key 1OS-F1-14
  misc_feature 1..58: note = A-key 1OS-F1-14
  source 1..58: mol_type = other DNA
ccatctcatccctgcgtgtctccgactcaggtcagagattctataaactgtgcggtcc

SEQ ID NO: 30 - DNA, 58 bp, synthetic construct
  misc_feature 1..58: note = A-key 1OS-F1-15
  misc_feature 1..58: note = A-key 1OS-F1-15
  source 1..58: mol_type = other DNA
ccatctcatccctgcgtgtctccgactcagcgagttgattctataaactgtgcggtcc

SEQ ID NO: 31 - DNA, 54 bp, synthetic construct
  misc_feature 1..54: note = A-key 2OS-F1-1
  misc_feature 1..54: note = A-key 2OS-F1-1
  source 1..54: mol_type = other DNA
ccatctcatccctgcgtgtctccgactcagctgggggaagttccagccagcgtc

SEQ ID NO: 32 - DNA, 54 bp, synthetic construct
  misc_feature 1..54: note = A-key 2OS-F1-2
  misc_feature 1..54: note = A-key 2OS-F1-2
  source 1..54: mol_type = other DNA
ccatctcatccctgcgtgtctccgactcagctccacgaagttccagccagcgtc

SEQ ID NO: 33 - DNA, 54 bp, synthetic construct
  misc_feature 1..54: note = A-key 2OS-F1-3
  misc_feature 1..54: note = A-key 2OS-F1-3
  source 1..54: mol_type = other DNA
ccatctcatccctgcgtgtctccgactcagcttaccgaagttccagccagcgtc

SEQ ID NO: 34 - DNA, 54 bp, synthetic construct
  misc_feature 1..54: note = A-key 2OS-F1-4
  misc_feature 1..54: note = A-key 2OS-F1-4
  source 1..54: mol_type = other DNA
ccatctcatccctgcgtgtctccgactcagtggcaggaagttccagccagcgtc

SEQ ID NO: 35 - DNA, 54 bp, synthetic construct
  misc_feature 1..54: note = A-key 2OS-F1-5
  misc_feature 1..54: note = A-key 2OS-F1-5
  source 1..54: mol_type = other DNA
ccatctcatccctgcgtgtctccgactcagtgagtagaagttccagccagcgtc

SEQ ID NO: 36 - DNA, 54 bp, synthetic construct
  misc_feature 1..54: note = A-key 2OS-F1-6
  misc_feature 1..54: note = A-key 2OS-F1-6
  source 1..54: mol_type = other DNA
ccatctcatccctgcgtgtctccgactcagattcaggaagttccagccagcgtc

SEQ ID NO: 37 - DNA, 54 bp, synthetic construct
  misc_feature 1..54: note = A-key 2OS-F1-7
  misc_feature 1..54: note = A-key 2OS-F1-7
  source 1..54: mol_type = other DNA
ccatctcatccctgcgtgtctccgactcagtgagctgaagttccagccagcgtc

SEQ ID NO: 38 - DNA, 54 bp, synthetic construct
  misc_feature 1..54: note = A-key 2OS-F1-8
  misc_feature 1..54: note = A-key 2OS-F1-8
  source 1..54: mol_type = other DNA
ccatctcatccctgcgtgtctccgactcagggcgtggaagttccagccagcgtc

SEQ ID NO: 39 - DNA, 54 bp, synthetic construct
  misc_feature 1..54: note = A-key 2OS-F1-9
  misc_feature 1..54: note = A-key 2OS-F1-9
  source 1..54: mol_type = other DNA
ccatctcatccctgcgtgtctccgactcagaaattggaagttccagccagcgtc

SEQ ID NO: 40 - DNA, 54 bp, synthetic construct
  misc_feature 1..54: note = A-key 2OS-F1-10
  misc_feature 1..54: note = A-key 2OS-F1-10
  source 1..54: mol_type = other DNA
ccatctcatccctgcgtgtctccgactcaggctgacgaagttccagccagcgtc

SEQ ID NO: 41 - DNA, 54 bp, synthetic construct
  misc_feature 1..54: note = A-key 2OS-F1-11
  misc_feature 1..54: note = A-key 2OS-F1-11
  source 1..54: mol_type = other DNA
ccatctcatccctgcgtgtctccgactcagttcttagaagttccagccagcgtc

SEQ ID NO: 42 - DNA, 54 bp, synthetic construct
  misc_feature 1..54: note = A-key 2OS-F1-12
  misc_feature 1..54: note = A-key 2OS-F1-12
  source 1..54: mol_type = other DNA
ccatctcatccctgcgtgtctccgactcagtggtgggaagttccagccagcgtc

SEQ ID NO: 43 - DNA, 54 bp, synthetic construct
  misc_feature 1..54: note = A-key 2OS-F1-13
  misc_feature 1..54: note = A-key 2OS-F1-13
  source 1..54: mol_type = other DNA
ccatctcatccctgcgtgtctccgactcaggcagtcgaagttccagccagcgtc

SEQ ID NO: 44 - DNA, 54 bp, synthetic construct
  misc_feature 1..54: note = A-key 2OS-F1-14
  misc_feature 1..54: note = A-key 2OS-F1-14
  source 1..54: mol_type = other DNA
ccatctcatccctgcgtgtctccgactcagtcgtgagaagttccagccagcgtc

SEQ ID NO: 45 - DNA, 54 bp, synthetic construct
  misc_feature 1..54: note = A-key 2OS-F1-15
  misc_feature 1..54: note = A-key 2OS-F1-15
  source 1..54: mol_type = other DNA
ccatctcatccctgcgtgtctccgactcagtacagtgaagttccagccagcgtc

SEQ ID NO: 46 - DNA, 44 bp, synthetic construct
  misc_feature 1..44: note = P1-key 1OS-R1
  misc_feature 1..44: note = P1-key 1OS-R1
  source 1..44: mol_type = other DNA
cctctctatgggcagtcggtgatgagtacatgatagcgccgtac

SEQ ID NO: 47 - DNA, 25 bp, synthetic construct
  misc_feature 1..25: note = Probe123, 6-FAM in 5', BHQ-1 in 3'
  misc_feature 1..25: note = Probe123
  source 1..25: mol_type = other DNA
gcctgtagtcccacgcgatctaaca

SEQ ID NO: 48 - DNA, 25 bp, synthetic construct
  misc_feature 1..25: note = Artificial sequence
  misc_feature 1..25: note = Probe124, HEX in 5', BHQ-1 in 3'
  source 1..25: mol_type = other DNA
caaccattgattggggacaactggg

SEQ ID NO: 49 - DNA, 18 bp, synthetic construct
  misc_feature 1..18: note = Forward primer
  primer_bind 1..18: note = Forward primer
  source 1..18: mol_type = other DNA
gaagttccagccagcgtc

SEQ ID NO: 50 - DNA, 21 bp, synthetic construct
  misc_feature 1..21: note = Reverse primer
  primer_bind 1..21: note = Reverse primer
  source 1..21: mol_type = other DNA
ctgtgactatgtgaggctttc

SEQ ID NO: 51 - DNA, 72 bp, synthetic construct
  misc_feature 1..72: note = 2OS-1-Oligo-A1, Biotin-C6 in 5'
  misc_feature 1..72: note = 2OS-1-Oligo-A1
  misc_feature 26..31: note = n: any of A, T, G, C independently
  source 1..72: mol_type = other DNA
gaagttccagccagcgtcacagtttnnnnnncgagggcaatggttaactgacacgtggtcagcatcatttcc

SEQ ID NO: 52 - DNA, 72 bp, synthetic construct
  misc_feature 1..72: note = 2OS-1-Oligo-A2, Biotin-C6 in 5'
  misc_feature 1..72: note = 2OS-1-Oligo-A1
  misc_feature 26..31: note = n: any of A, T, G, C independently
  source 1..72: mol_type = other DNA
gaagttccagccagcgtcacagtttnnnnnncagaaagcagtctcgtcggttcgaaggtcagcatcatttcc

SEQ ID NO: 53 - DNA, 72 bp, synthetic construct
  misc_feature 1..72: note = 2OS-1-Oligo-A3, Biotin-C6 in 5'
  misc_feature 1..72: note = 2OS-1-Oligo-A3
  misc_feature 26..31: note = n: any of A, T, G, C independently
  source 1..72: mol_type = other DNA
gaagttccagccagcgtcacagtttnnnnnntaagtagcgggcataatgtacgctcggtcagcatcatttcc

SEQ ID NO: 54 - DNA, 72 bp, synthetic construct
  misc_feature 1..72: note = 2OS-1-Oligo-A4, Biotin-C6 in 5'
  misc_feature 1..72: note = 2OS-1-Oligo-A4, Biotin-C6 in 5'
  misc_feature 26..31: note = n: any of A, T, G, C independently
  source 1..72: mol_type = other DNA
gaagttccagccagcgtcacagtttnnnnnnggatccagtaagctactgcgtttatggtcagcatcatttcc

SEQ ID NO: 55 - DNA, 72 bp, synthetic construct
  misc_feature 1..72: note = 2OS-1-Oligo-A5, Biotin-C6 in 5'
  misc_feature 1..72: note = 2OS-1-Oligo-A5
  misc_feature 26..31: note = n: any of A, T, G, C independently
  source 1..72: mol_type = other DNA
gaagttccagccagcgtcacagtttnnnnnngggctgcggagcgtttactctgtatggtcagcatcatttcc

SEQ ID NO: 56 - DNA, 72 bp, synthetic construct
  misc_feature 1..72: note = 2OS-1-Oligo-A6, Biotin-C6 in 5'
  misc_feature 1..72: note = 2OS-1-Oligo-A6
  misc_feature 26..31: note = n: any of A, T, G, C independently
  source 1..72: mol_type = other DNA
gaagttccagccagcgtcacagtttnnnnnnaaacgtatgtgctttgtcggatgccggtcagcatcatttcc

SEQ ID NO: 57 - DNA, 72 bp, synthetic construct
  misc_feature 1..72: note = 2OS-1-Oligo-A7, Biotin-C6 in 5'
  misc_feature 1..72: note = 2OS-1-Oligo-A7
  misc_feature 26..31: note = n: any of A, T, G, C independently
  source 1..72: mol_type = other DNA
gaagttccagccagcgtcacagtttnnnnnnatatcatcataggcttagcgacgtaggtcagcatcatttcc

SEQ ID NO: 58 - DNA, 72 bp, synthetic construct
  misc_feature 1..72: note = 2OS-1-Oligo-A8, Biotin-C6 in 5'
  misc_feature 1..72: note = 2OS-1-Oligo-A8
  misc_feature 26..31: note = n: any of A, T, G, C
  source 1..72: mol_type = other DNA
gaagttccagccagcgtcacagtttnnnnnnaggaaaatctgctaccgccaatgatggtcagcatcatttcc

SEQ ID NO: 59 - DNA, 72 bp, synthetic construct
  misc_feature 1..72: note = 2OS-1-Oligo-A9, Biotin-C6 in 5'
  misc_feature 1..72: note = 2OS-1-Oligo-A9
  misc_feature 26..31: note = n: any of A, T, G, C independently
  source 1..72: mol_type = other DNA
gaagttccagccagcgtcacagtttnnnnnnctgattgactgcatggaggctatacggtcagcatcatttcc

SEQ ID NO: 60 - DNA, 72 bp, synthetic construct
  misc_feature 1..72: note = 2OS-1-Oligo-A10, Biotin-C6 in 5'
  misc_feature 1..72: note = 2OS-1-Oligo-A10, Biotin-C6 in 5'
  misc_feature 26..31: note = n: any of A, T, G, C independently
  source 1..72: mol_type = other DNA
gaagttccagccagcgtcacagtttnnnnnngtggcgacttcacgattatctgaacggtcagcatcatttcc

SEQ ID NO: 61 - DNA, 72 bp, synthetic construct
  misc_feature 1..72: note = 2OS-1-Oligo-A11, Biotin-C6 in 5'
  misc_feature 1..72: note = 2OS-1-Oligo-A11, Biotin-C6 in 5'
  misc_feature 26..31: note = n: any of A, T, G, C independently
  source 1..72: mol_type = other DNA
gaagttccagccagcgtcacagtttnnnnnncctgtattgaaggttcagtcctgttggtcagcatcatttcc

SEQ ID NO: 62 - DNA, 72 bp, synthetic construct
  misc_feature 1..72: note = 2OS-1-Oligo-A12, Biotin-C6 in 5'
  misc_feature 1..72: note = 2OS-1-Oligo-A12, Biotin-C6 in 5', n: any of A, T, G, C independently
  source 1..72: mol_type = other DNA
gaagttccagccagcgtcacagtttnnnnnnggctctataaggtttcctcaaaggtggtcagcatcatttcc

SEQ ID NO: 63 - DNA, 72 bp, synthetic construct
  misc_feature 1..72: note = 2OS-1-Oligo-A13, Biotin-C6 in 5'
  misc_feature 1..72: note = 2OS-1-Oligo-A13, Biotin-C6 in 5', n: any of A, T, G, C independently
  source 1..72: mol_type = other DNA
gaagttccagccagcgtcacagtttnnnnnnttgggagctttcctatgtacagtccggtcagcatcatttcc

SEQ ID NO: 64 - DNA, 72 bp, synthetic construct
  misc_feature 1..72: note = 2OS-1-Oligo-A14, Biotin-C6 in 5'
  misc_feature 1..72: note = 2OS-1-Oligo-A14; Biotin-C6 in 5'; n: any of A, T, G, C independently
  source 1..72: mol_type = other DNA
gaagttccagccagcgtcacagtttnnnnnnagagaatatgtcgctcccgttatgtggtcagcatcatttcc

SEQ ID NO: 65 - DNA, 72 bp, synthetic construct
  misc_feature 1..72: note = 2OS-1-Oligo-A15; Biotin-C6 in 5'
  misc_feature 1..72: note = 2OS-1-Oligo-A15; Biotin-C6 in 5'; n: any of A, T, G, C independently
  source 1..72: mol_type = other DNA
gaagttccagccagcgtcacagtttnnnnnngcagttagatatgcagttacctgacggtcagcatcatttcc

SEQ ID NO: 66 - DNA, 72 bp, synthetic construct
  misc_feature 1..72: note = 2OS-1-Oligo-A16
  misc_feature 1..72: note = 2OS-1-Oligo-A16; Biotin-C6 in 5'; n: any of A, T, G, C independently
  source 1..72: mol_type = other DNA
gaagttccagccagcgtcacagtttnnnnnncttcacccgaacatgcagtgttattggtcagcatcatttcc

SEQ ID NO: 67 - DNA, 72 bp, synthetic construct
  misc_feature 1..72: note = 2OS-1-Oligo-A17
  misc_feature 1..72: note = 2OS-1-Oligo-A17; Biotin-C6 in 5'; n: any of A, T, G, C independently
  source 1..72: mol_type = other DNA
gaagttccagccagcgtcacagtttnnnnnnaaagccgttgcagtatcgtctgagcggtcagcatcatttcc

SEQ ID NO: 68 - DNA, 72 bp, synthetic construct
  misc_feature 1..72: note = 2OS-1-Oligo-A18
  misc_feature 1..72: note = 2OS-1-Oligo-A18; Biotin-C6 in 5'; n: any of A, T, G, C independently
  source 1..72: mol_type = other DNA
gaagttccagccagcgtcacagtttnnnnnngctggatgttaataactgcggtccgggtcagcatcatttcc

SEQ ID NO: 69 - DNA, 72 bp, synthetic construct
  misc_feature 1..72: note = 2OS-1-Oligo-A19
  misc_feature 1..72: note = 2OS-1-Oligo-A19; Biotin-C6 in 5'; n: any of A, T, G, C independently
  source 1..72: mol_type = other DNA
gaagttccagccagcgtcacagtttnnnnnnacgagttgacatggacggatccctcggtcagcatcatttcc

SEQ ID NO: 70 - DNA, 72 bp, synthetic construct
  misc_feature 1..72: note = 2OS-1-Oligo-A20
  misc_feature 1..72: note = 2OS-1-Oligo-A20; Biotin-C6 in 5'; n: any of A, T, G, C independently
  source 1..72: mol_type = other DNA
gaagttccagccagcgtcacagtttnnnnnnttcatcactcattgttctgagtaggggtcagcatcatttcc

SEQ ID NO: 71 - DNA, 72 bp, synthetic construct
  misc_feature 1..72: note = 2OS-1-Oligo-A21
  misc_feature 1..72: note = 2OS-1-Oligo-A21; Biotin-C6 in 5'; n: any of A, T, G, C independently
  source 1..72: mol_type = other DNA
gaagttccagccagcgtcacagtttnnnnnnatgtttaatctaacttgatgcctccggtcagcatcatttcc

SEQ ID NO: 72 - DNA, 72 bp, synthetic construct
  misc_feature 1..72: note = 2OS-1-Oligo-A22
  misc_feature 1..72: note = 2OS-1-Oligo-A22; Biotin-C6 in 5'; n: any of A, T, G, C independently
  source 1..72: mol_type = other DNA
gaagttccagccagcgtcacagtttnnnnnntaatacgcctgaggtgttgggttgcggtcagcatcatttcc

SEQ ID NO: 73 - DNA, 72 bp, synthetic construct
  misc_feature 1..72: note = 2OS-1-Oligo-B1
  misc_feature 1..72: note = 2OS-1-Oligo-B1; n: any of A, T, G, C independently
  source 1..72: mol_type = other DNA
ctgtgactatgtgaggctttctcgannnnnngcctgtagtcccacgcgatctaacaggaaatgatgctgacc

SEQ ID NO: 74 - DNA, 72 bp, synthetic construct
  misc_feature 1..72: note = 2OS-1-Oligo-B2
  misc_feature 1..72: note = 2OS-1-Oligo-B2; n: any of A, T, G, C independently
  source 1..72: mol_type = other DNA
ctgtgactatgtgaggctttctcgannnnnncaaccattgattggggacaactgggggaaatgatgctgacc

SEQ ID NO: 75 - DNA, 72 bp, synthetic construct
  misc_feature 1..72: note = 2OS-1-Oligo-B3
  misc_feature 1..72: note = 2OS-1-Oligo-B3; n: any of A, T, G, C independently
  source 1..72: mol_type = other DNA
ctgtgactatgtgaggctttctcgannnnnnacgtttaagcatctgtactccagatggaaatgatgctgacc

SEQ ID NO: 76 - DNA, 72 bp, synthetic construct
  misc_feature 1..72: note = 2OS-1-Oligo-B4
  misc_feature 1..72: note = 2OS-1-Oligo-B4; n: any of A, T, G, C independently
  source 1..72: mol_type = other DNA
ctgtgactatgtgaggctttctcgannnnnngaattgaagccatcgtttcgcgcaaggaaatgatgctgacc

SEQ ID NO: 77 - DNA, 72 bp, synthetic construct
  misc_feature 1..72: note = 2OS-1-Oligo-B5
  misc_feature 1..72: note = 2OS-1-Oligo-B5; n: any of A, T, G, C independently
  source 1..72: mol_type = other DNA
ctgtgactatgtgaggctttctcgannnnnncgtagcttttgtagcgtctgagggcggaaatgatgctgacc

SEQ ID NO: 78 - DNA, 72 bp, synthetic construct
  misc_feature 1..72: note = 2OS-1-Oligo-B6
  misc_feature 1..72: note = 2OS-1-Oligo-B6; n: any of A, T, G, C independently
  source 1..72: mol_type = other DNA
ctgtgactatgtgaggctttctcgannnnnnaatcgtcagtccctgtttcgacatcggaaatgatgctgacc

SEQ ID NO: 79 - DNA, 72 bp, synthetic construct
  misc_feature 1..72: note = 2OS-1-Oligo-B7
  misc_feature 1..72: note = 2OS-1-Oligo-B7; n: any of A, T, G, C independently
  source 1..72: mol_type = other DNA
ctgtgactatgtgaggctttctcgannnnnncggtggtaggtgatacttctgtaccggaaatgatgctgacc

SEQ ID NO: 80 - DNA, 72 bp, synthetic construct
  misc_feature 1..72: note = 2OS-1-Oligo-B8
  misc_feature 1..72: note = 2OS-1-Oligo-B8; n: any of A, T, G, C independently
  source 1..72: mol_type = other DNA
ctgtgactatgtgaggctttctcgannnnnntgactatcggggcgtgacatgagctggaaatgatgctgacc

SEQ ID NO: 81 - DNA, 72 bp, synthetic construct
  misc_feature 1..72: note = 2OS-1-Oligo-B9
  misc_feature 1..72: note = 2OS-1-Oligo-B9; n: any of A, T, G, C independently
  source 1..72: mol_type = other DNA
ctgtgactatgtgaggctttctcgannnnnngttggtgaaactaccgacgctttacggaaatgatgctgacc

SEQ ID NO: 82 - DNA, 72 bp, synthetic construct
  misc_feature 1..72: note = 2OS-1-Oligo-B10
  misc_feature 1..72: note = 2OS-1-Oligo-B10; n: any of A, T, G, C independently
  source 1..72: mol_type = other DNA
ctgtgactatgtgaggctttctcgannnnnnaatggaggtgcaggaatactctcgtggaaatgatgctgacc

SEQ ID NO: 83 - DNA, 72 bp, synthetic construct
  misc_feature 1..72: note = 2OS-1-Oligo-B11
  misc_feature 1..72: note = 2OS-1-Oligo-B11; n: any of A, T, G, C independently
  source 1..72: mol_type = other DNA
ctgtgactatgtgaggctttctcgannnnnnaaaacgcaccacaactcggacgtgaggaaatgatgctgacc

SEQ ID NO: 84 - DNA, 72 bp, synthetic construct
  misc_feature 1..72: note = 2OS-1-Oligo-B12
  misc_feature 1..72: note = 2OS-1-Oligo-B12; n: any of A, T, G, C independently
  source 1..72: mol_type = other DNA
ctgtgactatgtgaggctttctcgannnnnngccatataagcacagcacgcaatccggaaatgatgctgacc

SEQ ID NO: 85 - DNA, 72 bp, synthetic construct
  misc_feature 1..72: note = 2OS-1-Oligo-B13
  misc_feature 1..72: note = 2OS-1-Oligo-B13; n: any of A, T, G, C independently
  source 1..72: mol_type = other DNA
ctgtgactatgtgaggctttctcgannnnnncctatgcgaacttggtttatcctgcggaaatgatgctgacc

SEQ ID NO: 86 - DNA, 72 bp, synthetic construct
  misc_feature 1..72: note = 2OS-1-Oligo-B14
  misc_feature 1..72: note = 2OS-1-Oligo-B14; n: any of A, T, G, C independently
  source 1..72: mol_type = other DNA
ctgtgactatgtgaggctttctcgannnnnnaagctgcgtatcctcgaactagcagggaaatgatgctgacc

SEQ ID NO: 87 - DNA, 72 bp, synthetic construct
  misc_feature 1..72: note = 2OS-1-Oligo-B15
  misc_feature 1..72: note = 2OS-1-Oligo-B15; n: any of A, T, G, C independently
  source 1..72: mol_type = other DNA
ctgtgactatgtgaggctttctcgannnnnnatggcgcagacattctgtagtcgcaggaaatgatgctgacc

SEQ ID NO: 88 - DNA, 72 bp, synthetic construct
  misc_feature 1..72: note = 2OS-1-Oligo-B16
  misc_feature 1..72: note = 2OS-1-Oligo-B16
  source 1..72: mol_type = other DNA
ctgtgactatgtgaggctttctcgannnnnncttatggactggttggggacaatccggaaatgatgctgacc

SEQ ID NO: 89 - DNA, 72 bp, synthetic construct
  misc_feature 1..72: note = 2OS-1-Oligo-B17
  misc_feature 1..72: note = 2OS-1-Oligo-B17; n: any of A, T, G, C independently
  source 1..72: mol_type = other DNA
ctgtgactatgtgaggctttctcgannnnnntgtccttccttacgaaatattggtcggaaatgatgctgacc

SEQ ID NO: 90 - DNA, 72 bp, synthetic construct
  misc_feature 1..72: note = 2OS-1-Oligo-B18
  misc_feature 1..72: note = 2OS-1-Oligo-B18; n: any of A, T, G, C independently
  source 1..72: mol_type = other DNA
ctgtgactatgtgaggctttctcgannnnnntgatgaaccaatcctccgatttcttggaaatgatgctgacc

SEQ ID NO: 91 - DNA, 72 bp, synthetic construct
  misc_feature 1..72: note = 2OS-1-Oligo-B19
  misc_feature 1..72: note = 2OS-1-Oligo-B19; n: any of A, T, G, C independently
  source 1..72: mol_type = other DNA
ctgtgactatgtgaggctttctcgannnnnnaccgaatgtgggccacgagtcattcggaaatgatgctgacc

SEQ ID NO: 92 - DNA, 72 bp, synthetic construct
  misc_feature 1..72: note = 2OS-1-Oligo-B20
  misc_feature 1..72: note = 2OS-1-Oligo-B20; n: any of A, T, G, C independently
  source 1..72: mol_type = other DNA
ctgtgactatgtgaggctttctcgannnnnncgggtgagcatataacttgcaattcggaaatgatgctgacc

SEQ ID NO: 93 - DNA, 72 bp, synthetic construct
  misc_feature 1..72: note = 2OS-1-Oligo-B21
  misc_feature 1..72: note = 2OS-1-Oligo-B21; n: any of A, T, G, C independently
  source 1..72: mol_type = other DNA
ctgtgactatgtgaggctttctcgannnnnnagaattgtgcttggggcgattcataggaaatgatgctgacc

SEQ ID NO: 94 - DNA, 72 bp, synthetic construct
  misc_feature 1..72: note = 2OS-1-Oligo-B22
  misc_feature 1..72: note = 2OS-1-Oligo-B22; n: any of A, T, G, C independently
  source 1..72: mol_type = other DNA
ctgtgactatgtgaggctttctcgannnnnnaattggtgacatgcttaactaccgtggaaatgatgctgacc

SEQ ID NO: 95 - DNA, 72 bp, synthetic construct
  misc_feature 1..72: note = 2OS-1-Oligo-B23
  misc_feature 1..72: note = 2OS-1-Oligo-B23; n: any of A, T, G, C independently
  source 1..72: mol_type = other DNA
ctgtgactatgtgaggctttctcgannnnnngagacgcctagaaagtgattaactcggaaatgatgctgacc

SEQ ID NO: 96 - DNA, 72 bp, synthetic construct
  misc_feature 1..72: note = 2OS-1-Oligo-B24
  misc_feature 1..72: note = 2OS-1-Oligo-B24; n: any of A, T, G, C independently
  source 1..72: mol_type = other DNA
ctgtgactatgtgaggctttctcgannnnnnattacagttacagtgctggtcgcagggaaatgatgctgacc

SEQ ID NO: 97 - DNA, 72 bp, synthetic construct
  misc_feature 1..72: note = 2OS-1-Oligo-B25
  misc_feature 1..72: note = 2OS-1-Oligo-B25; n: any of A, T, G, C independently
  source 1..72: mol_type = other DNA
ctgtgactatgtgaggctttctcgannnnnncgttacgttggtgggctcttggtacggaaatgatgctgacc

SEQ ID NO: 98 - DNA, 72 bp, synthetic construct
  misc_feature 1..72: note = 2OS-1-Oligo-B26
  misc_feature 1..72: note = 2OS-1-Oligo-B26; n: any of A, T, G, C independently
  source 1..72: mol_type = other DNA
ctgtgactatgtgaggctttctcgannnnnngttattatcggtgtcccgactagttggaaatgatgctgacc

SEQ ID NO: 99 - DNA, 72 bp, synthetic construct
  misc_feature 1..72: note = 2OS-1-Oligo-B27
  misc_feature 1..72: note = 2OS-1-Oligo-B27; n: any of A, T, G, C independently
  source 1..72: mol_type = other DNA
ctgtgactatgtgaggctttctcgannnnnnagaaatgattcccgagtcgccttttggaaatgatgctgacc

SEQ ID NO: 100 - DNA, 72 bp, synthetic construct
  misc_feature 1..72: note = 2OS-1-Oligo-B28
  misc_feature 1..72: note = 2OS-1-Oligo-B28; n: any of A, T, G, C independently
  source 1..72: mol_type = other DNA
ctgtgactatgtgaggctttctcgannnnnntgctctcggatgtggttctatggatggaaatgatgctgacc

SEQ ID NO: 101 - DNA, 72 bp, synthetic construct
  misc_feature 1..72: note = 2OS-1-Oligo-B29
  misc_feature 1..72: note = 2OS-1-Oligo-B29; n: any of A, T, G, C independently
  source 1..72: mol_type = other DNA
ctgtgactatgtgaggctttctcgannnnnngagttaaaaccgtcgccgtagcactggaaatgatgctgacc

SEQ ID NO: 102 - DNA, 72 bp, synthetic construct
  misc_feature 1..72: note = 2OS-1-Oligo-B30
  misc_feature 1..72: note = 2OS-1-Oligo-B30; n: any of A, T, G, C independently
  source 1..72: mol_type = other DNA
ctgtgactatgtgaggctttctcgannnnnntgtacgcgatagtactcgggtcctgggaaatgatgctgacc

SEQ ID NO: 103 - DNA, 72 bp, synthetic construct
  misc_feature 1..72: note = 2OS-1-Oligo-B31
  misc_feature 1..72: note = 2OS-1-Oligo-B31; n: any of A, T, G, C independently
  source 1..72: mol_type = other DNA
ctgtgactatgtgaggctttctcgannnnnnaacttacgcccagcaaggcattcatggaaatgatgctgacc

SEQ ID NO: 104 - DNA, 72 bp, synthetic construct
  misc_feature 1..72: note = 2OS-1-Oligo-B32
  misc_feature 1..72: note = 2OS-1-Oligo-B32; n: any of A, T, G, C independently
  source 1..72: mol_type = other DNA
ctgtgactatgtgaggctttctcgannnnnnagcatggcacaagaggagcacttcaggaaatgatgctgacc

SEQ ID NO: 105 - DNA, 72 bp, synthetic construct
  misc_feature 1..72: note = 2OS-1-Oligo-B33
  misc_feature 1..72: note = 2OS-1-Oligo-B33; n: any of A, T, G, C independently
  source 1..72: mol_type = other DNA
ctgtgactatgtgaggctttctcgannnnnncgatcgtgagtttgcagcgtgacgaggaaatgatgctgacc

SEQ ID NO: 106 - DNA, 72 bp, synthetic construct
  misc_feature 1..72: note = 2OS-1-Oligo-B34
  misc_feature 1..72: note = 2OS-1-Oligo-B34; n: any of A, T, G, C independently
  source 1..72: mol_type = other DNA
ctgtgactatgtgaggctttctcgannnnnnacagctccagcctccctttgtttgtggaaatgatgctgacc

SEQ ID NO: 107 - DNA, 72 bp, synthetic construct
  misc_feature 1..72: note = 2OS-1-Oligo-B35
  misc_feature 1..72: note = 2OS-1-Oligo-B35; n: any of A, T, G, C independently
  source 1..72: mol_type = other DNA
ctgtgactatgtgaggctttctcgannnnnnaaacctttgttcgggcgtctaccatggaaatgatgctgacc

SEQ ID NO: 108 - DNA, 72 bp, synthetic construct
  misc_feature 1..72: note = 2OS-1-Oligo-B36
  misc_feature 1..72: note = 2OS-1-Oligo-B36; n: any of A, T, G, C independently
  source 1..72: mol_type = other DNA
ctgtgactatgtgaggctttctcgannnnnntctttcaaaacagcgggagtcatcgggaaatgatgctgacc

SEQ ID NO: 109 - DNA, 72 bp, synthetic construct
  misc_feature 1..72: note = 2OS-1-Oligo-B37
  misc_feature 1..72: note = 2OS-1-Oligo-B37; n: any of A, T, G, C independently
  source 1..72: mol_type = other DNA
ctgtgactatgtgaggctttctcgannnnnngcggtttatccgaatctcacgctaaggaaatgatgctgacc

SEQ ID NO: 110 - DNA, 72 bp, synthetic construct
  misc_feature 1..72: note = 2OS-1-Oligo-B38
  misc_feature 1..72: note = 2OS-1-Oligo-B38; n: any of A, T, G, C independently
  source 1..72: mol_type = other DNA
ctgtgactatgtgaggctttctcgannnnnngcatatgctacaggctggggtgaacggaaatgatgctgacc

SEQ ID NO: 111 - DNA, 72 bp, synthetic construct
  misc_feature 1..72: note = 2OS-1-Oligo-B39
  misc_feature 1..72: note = 2OS-1-Oligo-B39; n: any of A, T, G, C independently
  source 1..72: mol_type = other DNA
ctgtgactatgtgaggctttctcgannnnnnggaggtctaaacgtccggagctattggaaatgatgctgacc

SEQ ID NO: 112 - DNA, 72 bp, synthetic construct
  misc_feature 1..72: note = 2OS-1-Oligo-B40
  misc_feature 1..72: note = 2OS-1-Oligo-B40; n: any of A, T, G, C independently
  source 1..72: mol_type = other DNA
ctgtgactatgtgaggctttctcgannnnnnaagaataagattgcgtgcgccttaaggaaatgatgctgacc

SEQ ID NO: 113 - DNA, 72 bp, synthetic construct
  misc_feature 1..72: note = 2OS-1-Oligo-B41
  misc_feature 1..72: note = 2OS-1-Oligo-B41; n: any of A, T, G, C independently
  source 1..72: mol_type = other DNA
ctgtgactatgtgaggctttctcgannnnnncatcatcgtcgtccaaatatgtgatggaaatgatgctgacc

SEQ ID NO: 114 - DNA, 72 bp, synthetic construct
  misc_feature 1..72: note = Artificial sequence
  misc_feature 1..72: note = 2OS-1-Oligo-B42; n: any of A, T, G, C independently
  source 1..72: mol_type = other DNA
ctgtgactatgtgaggctttctcgannnnnncacgtgtagctgtgggccaagtctaggaaatgatgctgacc

SEQ ID NO: 115 - DNA, 72 bp, synthetic construct
  misc_feature 1..72: note = Artificial sequence
  misc_feature 1..72: note = 2OS-1-Oligo-B43; n: any of A, T, G, C independently
  source 1..72: mol_type = other DNA
ctgtgactatgtgaggctttctcgannnnnncagttgtcaaatctccgcattggtaggaaatgatgctgacc

SEQ ID NO: 116 - DNA, 72 bp, synthetic construct
  misc_feature 1..72: note = Artificial sequence
  misc_feature 1..72: note = 2OS-1-Oligo-B44; n: any of A, T, G, C independently
  source 1..72: mol_type = other DNA
ctgtgactatgtgaggctttctcgannnnnnactggtaatgccattggtctaaatgggaaatgatgctgacc

SEQ ID NO: 117 - DNA, 72 bp, synthetic construct
  misc_feature 1..72: note = Artificial sequence
  misc_feature 1..72: note = 2OS-1-Oligo-B45; n: any of A, T, G, C independently
  source 1..72: mol_type = other DNA
ctgtgactatgtgaggctttctcgannnnnngtctttggtcgtaacgaatctccgtggaaatgatgctgacc

SEQ ID NO: 118 - DNA, 72 bp, synthetic construct
  misc_feature 1..72: note = Artificial sequence
  misc_feature 1..72: note = 2OS-1-Oligo-B46; n: any of A, T, G, C independently
  source 1..72: mol_type = other DNA
ctgtgactatgtgaggctttctcgannnnnncttaggcatgacggggttgtccatgggaaatgatgctgacc

SEQ ID NO: 119 - DNA, 72 bp, synthetic construct
  misc_feature 1..72: note = Artificial sequence
  misc_feature 1..72: note = 2OS-1-Oligo-B47; n: any of A, T, G, C independently
  source 1..72: mol_type = other DNA
ctgtgactatgtgaggctttctcgannnnnnccggtgaattttgggtgtccatgtaggaaatgatgctgacc

SEQ ID NO: 120 - DNA, 72 bp, synthetic construct
  misc_feature 1..72: note = Artificial sequence
  misc_feature 1..72: note = 2OS-1-Oligo-B48; n: any of A, T, G, C independently
  source 1..72: mol_type = other DNA
ctgtgactatgtgaggctttctcgannnnnncctttatctcctccacctataaggtggaaatgatgctgacc

SEQ ID NO: 121 - DNA, 72 bp, synthetic construct
  misc_feature 1..72: note = Artificial sequence
  misc_feature 1..72: note = 2OS-1-Oligo-B49; n: any of A, T, G, C independently
  source 1..72: mol_type = other DNA
ctgtgactatgtgaggctttctcgannnnnngatactatatgacggcctgtaatcgggaaatgatgctgacc

SEQ ID NO: 122 - DNA, 72 bp, synthetic construct
  misc_feature 1..72: note = Artificial sequence
  misc_feature 1..72: note = 2OS-1-Oligo-B50; n: any of A, T, G, C independently
  source 1..72: mol_type = other DNA
ctgtgactatgtgaggctttctcgannnnnnattggttggccgaaagactacatctggaaatgatgctgacc

SEQ ID NO: 123 - DNA, 72 bp, synthetic construct
  misc_feature 1..72: note = Artificial sequence
  misc_feature 1..72: note = 2OS-1-Oligo-B51; n: any of A, T, G, C independently
  source 1..72: mol_type = other DNA
ctgtgactatgtgaggctttctcgannnnnncgtagttatggggtgggtcacctgcggaaatgatgctgacc

SEQ ID NO: 124 - DNA, 72 bp, synthetic construct
  misc_feature 1..72: note = Artificial sequence
  misc_feature 1..72: note = 2OS-1-Oligo-B52; n: any of A, T, G, C independently
  source 1..72: mol_type = other DNA
ctgtgactatgtgaggctttctcgannnnnnaagtttccaggcactgattcgttccggaaatgatgctgacc

SEQ ID NO: 125 - DNA, 72 bp, synthetic construct
  misc_feature 1..72: note = Artificial sequence
  misc_feature 1..72: note = 2OS-1-Oligo-B53; n: any of A, T, G, C independently
  source 1..72: mol_type = other DNA
ctgtgactatgtgaggctttctcgannnnnnttccttatttcccggttgagatacaggaaatgatgctgacc

SEQ ID NO: 126 - DNA, 72 bp, synthetic construct
  misc_feature 1..72: note = Artificial sequence
  misc_feature 1..72: note = 2OS-1-Oligo-B54; n: any of A, T, G, C independently
  source 1..72: mol_type = other DNA
ctgtgactatgtgaggctttctcgannnnnnaggtatcatgcgggccgaatcttggggaaatgatgctgacc

SEQ ID NO: 127 - DNA, 72 bp, synthetic construct
  misc_feature 1..72: note = Artificial sequence
  misc_feature 1..72: note = 2OS-1-Oligo-B55; n: any of A, T, G, C independently
  source 1..72: mol_type = other DNA
ctgtgactatgtgaggctttctcgannnnnnatacccgtaggccagtaccctctccggaaatgatgctgacc

SEQ ID NO: 128 - DNA, 81 bp, synthetic construct
  misc_feature 1..81: note = Artificial sequence
  misc_feature 1..81: note = 1OS-1-Oligo-1; Biotin-C6 in 5'; n: any of A, T, G, C independently
  source 1..81: mol_type = other DNA
agattctataaactgtgcggtccttnnnnnntatgaggacgaatctcccgcttataggtacggcgctatcatgtactcatg

SEQ ID NO: 129 - DNA, 81 bp, synthetic construct
  misc_feature 1..81: note = Artificial sequence
  misc_feature 1..81: note = 1OS-1-Oligo-2; Biotin-C6 in 5'; n: any of A, T, G, C independently
  source 1..81: mol_type = other DNA
agattctataaactgtgcggtccttnnnnnnggtcttgacaaacgtgtgcttgtacggtacggcgctatcatgtactcatg

SEQ ID NO: 130 - DNA, 81 bp, synthetic construct
  misc_feature 1..81: note = Artificial sequence
  misc_feature 1..81: note = 1OS-1-Oligo-3; Biotin-C6 in 5'; n: any of A, T, G, C independently
  source 1..81: mol_type = other DNA
agattctataaactgtgcggtccttnnnnnngtttatcgggcgtggtgctcgcataggtacggcgctatcatgtactcatg

SEQ ID NO: 131 - DNA, 81 bp, synthetic construct
  misc_feature 1..81: note = Artificial sequence
  misc_feature 1..81: note = 1OS-1-Oligo-4; Biotin-C6 in 5'; n: any of A, T, G, C independently
  source 1..81: mol_type = other DNA
agattctataaactgtgcggtccttnnnnnnccgatgttgacggactaatcctgacggtacggcgctatcatgtactcatg

SEQ ID NO: 132 - DNA, 81 bp, synthetic construct
  misc_feature 1..81: note = Artificial sequence
  misc_feature 1..81: note = 1OS-1-Oligo-5; Biotin-C6 in 5'; n: any of A, T, G, C independently
  source 1..81: mol_type = other DNA
agattctataaactgtgcggtccttnnnnnntagtagttcagacgccgttaagcgcggtacggcgctatcatgtactcatg

SEQ ID NO: 133 - DNA, 81 bp, synthetic construct
  misc_feature 1..81: note = Artificial sequence
  misc_feature 1..81: note = 1OS-1-Oligo-6; Biotin-C6 in 5'; n: any of A, T, G, C independently
  source 1..81: mol_type = other DNA
agattctataaactgtgcggtccttnnnnnnccgtacctagatacactcaatttgtggtacggcgctatcatgtactcatg

SEQ ID NO: 134 - DNA, 81 bp, synthetic construct
  misc_feature 1..81: note = Artificial sequence
  misc_feature 1..81: note = 1OS-1-Oligo-7; Biotin-C6 in 5'; n: any of A, T, G, C independently
  source 1..81: mol_type = other DNA
agattctataaactgtgcggtccttnnnnnnggggttccgttttacattccaggaaggtacggcgctatcatgtactcatg

SEQ ID NO: 135 - DNA, 81 bp, synthetic construct
  misc_feature 1..81: note = Artificial sequence
  misc_feature 1..81: note = 1OS-1-Oligo-8: Biotin-C6 in 5'; n: any of A, T, G, C independently
  source 1..81: mol_type = other DNA
agattctataaactgtgcggtccttnnnnnntatcccgtgaagcttgagtggaatcggtacggcgctatcatgtactcatg

SEQ ID NO: 136 - DNA, 81 bp, synthetic construct
  misc_feature 1..81: note = Artificial sequence
  misc_feature 1..81: note = 1OS-1-Oligo-9; Biotin-C6 in 5'; n: any of A, T, G, C independently
  source 1..81: mol_type = other DNA
agattctataaactgtgcggtccttnnnnnnctgacgtgtgaggcgctagagcataggtacggcgctatcatgtactcatg

SEQ ID NO: 137 - DNA, 81 bp, synthetic construct
  misc_feature 1..81: note = Artificial sequence
  misc_feature 1..81: note = 1OS-1-Oligo-10; Biotin-C6 in 5'; n: any of A, T, G, C independently
  source 1..81: mol_type = other DNA
agattctataaactgtgcggtccttnnnnnnggtatggcacgcctaatctggacacggtacggcgctatcatgtactcatg

SEQ ID NO: 138 - DNA, 81 bp, synthetic construct
  misc_feature 1..81: note = Artificial sequence
  misc_feature 1..81: note = 1OS-1-Oligo-11; Biotin-C6 in 5'; n: any of A, T, G, C independently
  source 1..81: mol_type = other DNA
agattctataaactgtgcggtccttnnnnnnggatgcatgatctagggcctcgtctggtacggcgctatcatgtactcatg

SEQ ID NO: 139 - DNA, 81 bp, synthetic construct
  misc_feature 1..81: note = Artificial sequence
  misc_feature 1..81: note = 1OS-1-Oligo-12; Biotin-C6 in 5'; n: any of A, T, G, C independently
  source 1..81: mol_type = other DNA
agattctataaactgtgcggtccttnnnnnngaggtctttcatgcgtatagtcacaggtacggcgctatcatgtactcatg

SEQ ID NO: 140 - DNA, 81 bp, synthetic construct
  misc_feature 1..81: note = Artificial sequence
  misc_feature 1..81: note = 1OS-1-Oligo-13; Biotin-C6 in 5'; n: any of A, T, G, C independently
  source 1..81: mol_type = other DNA
agattctataaactgtgcggtccttnnnnnngattcaatatgtgtcgtctatcctcggtacggcgctatcatgtactcatg

SEQ ID NO: 141 - DNA, 81 bp, synthetic construct
  misc_feature 1..81: note = Artificial sequence
  misc_feature 1..81: note = 1OS-1-Oligo-14; Biotin-C6 in 5'; n: any of A, T, G, C independently
  source 1..81: mol_type = other DNA
agattctataaactgtgcggtccttnnnnnnggtaactgcgcatagttggctctatggtacggcgctatcatgtactcatg

SEQ ID NO: 142 - DNA, 81 bp, synthetic construct
  misc_feature 1..81: note = Artificial sequence
  misc_feature 1..81: note = 1OS-1-Oligo-15; Biotin-C6 in 5'; n: any of A, T, G, C independently
  source 1..81: mol_type = other DNA
agattctataaactgtgcggtccttnnnnnngcgtttaaggtcacatcgcatgaatggtacggcgctatcatgtactcatg

SEQ ID NO: 143 - DNA, 81 bp, synthetic construct
  misc_feature 1..81: note = Artificial sequence
  misc_feature 1..81: note = 1OS-1-Oligo-16; Biotin-C6 in 5'; n: any of A, T, G, C independently
  source 1..81: mol_type = other DNA
agattctataaactgtgcggtccttnnnnnngcccgggaagtgtgaggatatacccggtacggcgctatcatgtactcatg

SEQ ID NO: 144 - DNA, 81 bp, synthetic construct
  misc_feature 1..81: note = Artificial sequence
  misc_feature 1..81: note = 1OS-1-Oligo-17; Biotin-C6 in 5'; n: any of A, T, G, C independently
  source 1..81: mol_type = other DNA
agattctataaactgtgcggtccttnnnnnngctcttaaaactggtatcacctgacggtacggcgctatcatgtactcatg

SEQ ID NO: 145 - DNA, 81 bp, synthetic construct
  misc_feature 1..81: note = Artificial sequence
  misc_feature 1..81: note = 1OS-1-Oligo-18; Biotin-C6 in 5'; n: any of A, T, G, C independently
  source 1..81: mol_type = other DNA
agattctataaactgtgcggtccttnnnnnngggtggttagtgatttgcccgtcacggtacggcgctatcatgtactcatg

SEQ ID NO: 146 - DNA, 81 bp, synthetic construct
  misc_feature 1..81: note = Artificial sequence
  misc_feature 1..81: note = 1OS-1-Oligo-19; Biotin-C6 in 5'; n: any of A, T, G, C independently
  source 1..81: mol_type = other DNA
agattctataaactgtgcggtccttnnnnnntagttggtgggtttccctaccgtgtggtacggcgctatcatgtactcatg

SEQ ID NO: 147 - DNA, 81 bp, synthetic construct
  misc_feature 1..81: note = Artificial sequence
  misc_feature 1..81: note = 1OS-1-Oligo-20; Biotin-C6 in 5'; n: any of A, T, G, C independently
  source 1..81: mol_type = other DNA
agattctataaactgtgcggtccttnnnnnnggtacagtaagtgagaatcctctctggtacggcgctatcatgtactcatg

SEQ ID NO: 148 - DNA, 81 bp, synthetic construct
  misc_feature 1..81: note = Artificial sequence
  misc_feature 1..81: note = 1OS-1-Oligo-21; Biotin-C6 in 5'; n: any of A, T, G, C independently
  source 1..81: mol_type = other DNA
agattctataaactgtgcggtccttnnnnnnggttctaagtttagcgtagccggttggtacggcgctatcatgtactcatg

SEQ ID NO: 149 - DNA, 81 bp, synthetic construct
  misc_feature 1..81: note = Artificial sequence
  misc_feature 1..81: note = 1OS-1-Oligo-22; Biotin-C6 in 5'; n: any of A, T, G, C independently
  source 1..81: mol_type = other DNA
agattctataaactgtgcggtccttnnnnnnctttaggtgggtgcgattgccagttggtacggcgctatcatgtactcatg

SEQ ID NO: 150 - DNA, 81 bp, synthetic construct
  misc_feature 1..81: note = Artificial sequence
  misc_feature 1..81: note = 1OS-1-Oligo-23; Biotin-C6 in 5'; n: any of A, T, G, C independently
  source 1..81: mol_type = other DNA
agattctataaactgtgcggtccttnnnnnngccaccttaacacgcgatgatattgggtacggcgctatcatgtactcatg

SEQ ID NO: 151 - DNA, 81 bp, synthetic construct
  misc_feature 1..81: note = Artificial sequence
  misc_feature 1..81: note = 1OS-1-Oligo-24; Biotin-C6 in 5'; n: any of A, T, G, C independently
  source 1..81: mol_type = other DNA
agattctataaactgtgcggtccttnnnnnngctattacgagcgcttggatcccgtggtacggcgctatcatgtactcatg

SEQ ID NO: 152 - DNA, 81 bp, synthetic construct
  misc_feature 1..81: note = Artificial sequence
  misc_feature 1..81: note = 1OS-1-Oligo-25; Biotin-C6 in 5'; n: any of A, T, G, C independently
  source 1..81: mol_type = other DNA
agattctataaactgtgcggtccttnnnnnntatgttgtgccttacgcctcgattaggtacggcgctatcatgtactcatg

SEQ ID NO: 153 - DNA, 81 bp, synthetic construct
  misc_feature 1..81: note = Artificial sequence
  misc_feature 1..81: note = 1OS-1-Oligo-26; Biotin-C6 in 5'; n: any of A, T, G, C independently
  source 1..81: mol_type = other DNA
agattctataaactgtgcggtccttnnnnnnttaaccgaactgacggccatcaaggggtacggcgctatcatgtactcatg

SEQ ID NO: 154 - DNA, 81 bp, synthetic construct
  misc_feature 1..81: note = Artificial sequence
  misc_feature 1..81: note = 1OS-1-Oligo-27 ; Biotin-C6 in 5'; n: any of A, T, G, C independently
  source 1..81: mol_type = other DNA
agattctataaactgtgcggtccttnnnnnngggtacatgcgccttactccttgtgggtacggcgctatcatgtactcatg

SEQ ID NO: 155 - DNA, 81 bp, synthetic construct
  misc_feature 1..81: note = Artificial sequence
  misc_feature 1..81: note = 1OS-1-Oligo-28; Biotin-C6 in 5'; n: any of A, T, G, C independently
  source 1..81: mol_type = other DNA
agattctataaactgtgcggtccttnnnnnnttctattctaagccggcggtcatatggtacggcgctatcatgtactcatg

SEQ ID NO: 156 - DNA, 81 bp, synthetic construct
  misc_feature 1..81: note = Artificial sequence
  misc_feature 1..81: note = 1OS-1-Oligo-29; Biotin-C6 in 5'; n: any of A, T, G, C independently
  source 1..81: mol_type = other DNA
agattctataaactgtgcggtccttnnnnnngcttgatgctttacaagatcgcgttggtacggcgctatcatgtactcatg

SEQ ID NO: 157 - DNA, 81 bp, synthetic construct
  misc_feature 1..81: note = Artificial sequence
  misc_feature 1..81: note = 1OS-1-Oligo-30; Biotin-C6 in 5'; n: any of A, T, G, C independently
  source 1..81: mol_type = other DNA
agattctataaactgtgcggtccttnnnnnntccaagttagcttactccatgccccggtacggcgctatcatgtactcatg

SEQ ID NO: 158 - DNA, 81 bp, synthetic construct
  misc_feature 1..81: note = Artificial sequence
  misc_feature 1..81: note = 1OS-1-Oligo-31; Biotin-C6 in 5'; n: any of A, T, G, C independently
  source 1..81: mol_type = other DNA
agattctataaactgtgcggtccttnnnnnnagaactatttcctggctgttacgcgggtacggcgctatcatgtactcatg

SEQ ID NO: 159 - DNA, 81 bp, synthetic construct
  misc_feature 1..81: note = Artificial sequence
  misc_feature 1..81: note = 1OS-1-Oligo-32; Biotin-C6 in 5'; n: any of A, T, G, C independently
  source 1..81: mol_type = other DNA
agattctataaactgtgcggtccttnnnnnntcggtttcaaggatgatccgcgcttggtacggcgctatcatgtactcatg

SEQ ID NO: 160 - DNA, 81 bp, synthetic construct
  misc_feature 1..81: note = Artificial sequence
  misc_feature 1..81: note = 1OS-1-Oligo-33; Biotin-C6 in 5'; n: any of A, T, G, C independently
  source 1..81: mol_type = other DNA
agattctataaactgtgcggtccttnnnnnnagagactgcccgacacatcttagtgggtacggcgctatcatgtactcatg

SEQ ID NO: 161 - DNA, 81 bp, synthetic construct
  misc_feature 1..81: note = Artificial sequence
  misc_feature 1..81: note = 1OS-1-Oligo-34 ; Biotin-C6 in 5'; n: any of A, T, G, C independently
  source 1..81: mol_type = other DNA
agattctataaactgtgcggtccttnnnnnnctgttaattaggctcggtcggcctaggtacggcgctatcatgtactcatg

SEQ ID NO: 162 - DNA, 81 bp, synthetic construct
  misc_feature 1..81: note = Artificial sequence
  misc_feature 1..81: note = 1OS-1-Oligo-35; Biotin-C6 in 5'; n: any of A, T, G, C independently
  source 1..81: mol_type = other DNA
agattctataaactgtgcggtccttnnnnnnaggtagtcctatgcgggctttctctggtacggcgctatcatgtactcatg

SEQ ID NO: 163 - DNA, 81 bp, synthetic construct
  misc_feature 1..81: note = Artificial sequence
  misc_feature 1..81: note = 1OS-1-Oligo-36; Biotin-C6 in 5'; n: any of A, T, G, C independently
  source 1..81: mol_type = other DNA
agattctataaactgtgcggtccttnnnnnnggcttggactatagtcatcgcgtttggtacggcgctatcatgtactcatg

SEQ ID NO: 164 - DNA, 81 bp, synthetic construct
  misc_feature 1..81: note = Artificial sequence
  misc_feature 1..81: note = 1OS-1-Oligo-37; Biotin-C6 in 5'; n: any of A, T, G, C independently
  source 1..81: mol_type = other DNA
agattctataaactgtgcggtccttnnnnnncactgtttaacaagcccgtcagtagggtacggcgctatcatgtactcatg

SEQ ID NO: 165 - DNA, 81 bp, synthetic construct
  misc_feature 1..81: note = Artificial sequence
  misc_feature 1..81: note = 1OS-1-Oligo-38; Biotin-C6 in 5'; n: any of A, T, G, C independently
  source 1..81: mol_type = other DNA
agattctataaactgtgcggtccttnnnnnnacgtcgtattatacccgccatggaaggtacggcgctatcatgtactcatg

SEQ ID NO: 166 - DNA, 81 bp, synthetic construct
  misc_feature 1..81: note = Artificial sequence
  misc_feature 1..81: note = 1OS-1-Oligo-39; Biotin-C6 in 5'; n: any of A, T, G, C independently
  source 1..81: mol_type = other DNA
agattctataaactgtgcggtccttnnnnnntgcttaatttacgaccgatgctgcgggtacggcgctatcatgtactcatg

SEQ ID NO: 167 - DNA, 81 bp, synthetic construct
  misc_feature 1..81: note = Artificial sequence
  misc_feature 1..81: note = 1OS-1-Oligo-40; Biotin-C6 in 5'; n: any of A, T, G, C independently
  source 1..81: mol_type = other DNA
agattctataaactgtgcggtccttnnnnnntccatagatttctccgtgagtctttggtacggcgctatcatgtactcatg

SEQ ID NO: 168 - DNA, 81 bp, synthetic construct
  misc_feature 1..81: note = Artificial sequence
  misc_feature 1..81: note = 1OS-1-Oligo-41; Biotin-C6 in 5'; n: any of A, T, G, C independently
  source 1..81: mol_type = other DNA
agattctataaactgtgcggtccttnnnnnngtgccgcagacattgcatacgatatggtacggcgctatcatgtactcatg

SEQ ID NO: 169 - DNA, 81 bp, synthetic construct
  misc_feature 1..81: note = Artificial sequence
  misc_feature 1..81: note = 1OS-1-Oligo-42; Biotin-C6 in 5'; n: any of A, T, G, C independently
  source 1..81: mol_type = other DNA
agattctataaactgtgcggtccttnnnnnngcaggtcctaacccgcaaccatttaggtacggcgctatcatgtactcatg

SEQ ID NO: 170 - DNA, 81 bp, synthetic construct
  misc_feature 1..81: note = Artificial sequence
  misc_feature 1..81: note = 1OS-1-Oligo-43; Biotin-C6 in 5'; n: any of A, T, G, C independently
  source 1..81: mol_type = other DNA
agattctataaactgtgcggtccttnnnnnntgcaccgttcatatgttatcgggacggtacggcgctatcatgtactcatg

SEQ ID NO: 171 - DNA, 81 bp, synthetic construct
  misc_feature 1..81: note = Artificial sequence
  misc_feature 1..81: note = 1OS-1-Oligo-44; Biotin-C6 in 5'; n: any of A, T, G, C independently
  source 1..81: mol_type = other DNA
agattctataaactgtgcggtccttnnnnnnagagacttacacccgtagacgtcggggtacggcgctatcatgtactcatg

SEQ ID NO: 172 - DNA, 81 bp, synthetic construct
  misc_feature 1..81: note = Artificial sequence
  misc_feature 1..81: note = 1OS-1-Oligo-45; Biotin-C6 in 5'; n: any of A, T, G, C independently
  source 1..81: mol_type = other DNA
agattctataaactgtgcggtccttnnnnnnataaaagaaaccctccgcattgtgtggtacggcgctatcatgtactcatg

SEQ ID NO: 173 - DNA, 81 bp, synthetic construct
  misc_feature 1..81: note = Artificial sequence
  misc_feature 1..81: note = 1OS-1-Oligo-46; Biotin-C6 in 5'; n: any of A, T, G, C independently
  source 1..81: mol_type = other DNA
agattctataaactgtgcggtccttnnnnnnggtcccatccgagcagatttgactcggtacggcgctatcatgtactcatg

SEQ ID NO: 174 - DNA, 81 bp, synthetic construct
  misc_feature 1..81: note = Artificial sequence
  misc_feature 1..81: note = 1OS-1-Oligo-47; Biotin-C6 in 5'; n: any of A, T, G, C independently
  source 1..81: mol_type = other DNA
agattctataaactgtgcggtccttnnnnnnatgagctgtctcgaaccgaaggcacggtacggcgctatcatgtactcatg

SEQ ID NO: 175 - DNA, 81 bp, synthetic construct
  misc_feature 1..81: note = Artificial sequence
  misc_feature 1..81: note = 1OS-1-Oligo-48; Biotin-C6 in 5'; n: any of A, T, G, C independently
  source 1..81: mol_type = other DNA
agattctataaactgtgcggtccttnnnnnntcgggcggttcaacttactggtagaggtacggcgctatcatgtactcatg

SEQ ID NO: 176 - DNA, 81 bp, synthetic construct
  misc_feature 1..81: note = Artificial sequence
  misc_feature 1..81: note = 1OS-1-Oligo-49; Biotin-C6 in 5'; n: any of A, T, G, C independently
  source 1..81: mol_type = other DNA
agattctataaactgtgcggtccttnnnnnnggggaaataacggatgcgctcttgaggtacggcgctatcatgtactcatg

SEQ ID NO: 177 - DNA, 81 bp, synthetic construct
  misc_feature 1..81: note = Artificial sequence
  misc_feature 1..81: note = 1OS-1-Oligo-50; Biotin-C6 in 5'; n: any of A, T, G, C independently
  source 1..81: mol_type = other DNA
agattctataaactgtgcggtccttnnnnnnacttcttctcggtcgcatgaggctgggtacggcgctatcatgtactcatg

SEQ ID NO: 178 - DNA, 81 bp, synthetic construct
  misc_feature 1..81: note = Artificial sequence
  misc_feature 1..81: note = 1OS-1-Oligo-51; Biotin-C6 in 5'; n: any of A, T, G, C independently
  source 1..81: mol_type = other DNA
agattctataaactgtgcggtccttnnnnnnggatacatatacgctcgtcgggactggtacggcgctatcatgtactcatg

SEQ ID NO: 179 - DNA, 81 bp, synthetic construct
  misc_feature 1..81: note = Artificial sequence
  misc_feature 1..81: note = 1OS-1-Oligo-52; Biotin-C6 in 5'; n: any of A, T, G, C independently
  source 1..81: mol_type = other DNA
agattctataaactgtgcggtccttnnnnnnccgggaagtgtcataacttgaagcgggtacggcgctatcatgtactcatg

SEQ ID NO: 180 - DNA, 81 bp, synthetic construct
  misc_feature 1..81: note = Artificial sequence
  misc_feature 1..81: note = 1OS-1-Oligo-53; Biotin-C6 in 5'; n: any of A, T, G, C independently
  source 1..81: mol_type = other DNA
agattctataaactgtgcggtccttnnnnnnctcagcctgcctcgcttctgatattggtacggcgctatcatgtactcatg

SEQ ID NO: 181 - DNA, 81 bp, synthetic construct
  misc_feature 1..81: note = Artificial sequence
  misc_feature 1..81: note = 1OS-1-Oligo-54; Biotin-C6 in 5'; n: any of A, T, G, C independently
  source 1..81: mol_type = other DNA
agattctataaactgtgcggtccttnnnnnnagggccaagtcgacctagatggctaggtacggcgctatcatgtactcatg

SEQ ID NO: 182 - DNA, 81 bp, synthetic construct
  misc_feature 1..81: note = Artificial sequence
  misc_feature 1..81: note = 1OS-1-Oligo-55; Biotin-C6 in 5'; n: any of A, T, G, C independently
  source 1..81: mol_type = other DNA
agattctataaactgtgcggtccttnnnnnnggtagggctactgttatcctccgtcggtacggcgctatcatgtactcatg

SEQ ID NO: 183 - DNA, 81 bp, synthetic construct
  misc_feature 1..81: note = Artificial sequence
  misc_feature 1..81: note = 1OS-1-Oligo-56; Biotin-C6 in 5'; n: any of A, T, G, C independently
  source 1..81: mol_type = other DNA
agattctataaactgtgcggtccttnnnnnncgtacggctggagagctgtatgtggggtacggcgctatcatgtactcatg

SEQ ID NO: 184 - DNA, 81 bp, synthetic construct
  misc_feature 1..81: note = Artificial sequence
  misc_feature 1..81: note = 1OS-1-Oligo-57; Biotin-C6 in 5'; n: any of A, T, G, C independently
  source 1..81: mol_type = other DNA
agattctataaactgtgcggtccttnnnnnnacaggttgtattacttcgcgccttgggtacggcgctatcatgtactcatg

SEQ ID NO: 185 - DNA, 81 bp, synthetic construct
  misc_feature 1..81: note = Artificial sequence
  misc_feature 1..81: note = 1OS-1-Oligo-58; Biotin-C6 in 5'; n: any of A, T, G, C independently
  source 1..81: mol_type = other DNA
agattctataaactgtgcggtccttnnnnnnctgggctcattacaagtgttgcataggtacggcgctatcatgtactcatg

SEQ ID NO: 186 - DNA, 81 bp, synthetic construct
  misc_feature 1..81: note = Artificial sequence
  misc_feature 1..81: note = 1OS-1-Oligo-59; Biotin-C6 in 5'; n: any of A, T, G, C independently
  source 1..81: mol_type = other DNA
agattctataaactgtgcggtccttnnnnnnctaagtggcgccgattgtttgtccaggtacggcgctatcatgtactcatg

SEQ ID NO: 187 - DNA, 81 bp, synthetic construct
  misc_feature 1..81: note = Artificial sequence
  misc_feature 1..81: note = 1OS-1-Oligo-60; Biotin-C6 in 5'; n: any of A, T, G, C independently
  source 1..81: mol_type = other DNA
agattctataaactgtgcggtccttnnnnnngtatattttgctcccggcgacgagaggtacggcgctatcatgtactcatg

SEQ ID NO: 188 - DNA, 81 bp, synthetic construct
  misc_feature 1..81: note = Artificial sequence
  misc_feature 1..81: note = 1OS-1-Oligo-61; Biotin-C6 in 5'; n: any of A, T, G, C independently
  source 1..81: mol_type = other DNA
agattctataaactgtgcggtccttnnnnnngcaatttgcgcttgttcggcatagcggtacggcgctatcatgtactcatg

SEQ ID NO: 189 - DNA, 81 bp, synthetic construct
  misc_feature 1..81: note = Artificial sequence
  misc_feature 1..81: note = 1OS-1-Oligo-62; Biotin-C6 in 5'; n: any of A, T, G, C independently
  source 1..81: mol_type = other DNA
agattctataaactgtgcggtccttnnnnnngagtcgaatatccaccaccgtatggggtacggcgctatcatgtactcatg

SEQ ID NO: 190 - DNA, 81 bp, synthetic construct
  misc_feature 1..81: note = Artificial sequence
  misc_feature 1..81: note = 1OS-1-Oligo-63; Biotin-C6 in 5'; n: any of A, T, G, C independently
  source 1..81: mol_type = other DNA
agattctataaactgtgcggtccttnnnnnnttgtggtttgggtcctcagaggagaggtacggcgctatcatgtactcatg

SEQ ID NO: 191 - DNA, 81 bp, synthetic construct
  misc_feature 1..81: note = Artificial sequence
  misc_feature 1..81: note = 1OS-1-Oligo-64; Biotin-C6 in 5'; n: any of A, T, G, C independently
  source 1..81: mol_type = other DNA
agattctataaactgtgcggtccttnnnnnnggtacctagtctcgtaatcataggaggtacggcgctatcatgtactcatg

SEQ ID NO: 192 - DNA, 81 bp, synthetic construct
  misc_feature 1..81: note = Artificial sequence
  misc_feature 1..81: note = 1OS-1-Oligo-65; Biotin-C6 in 5'; n: any of A, T, G, C independently
  source 1..81: mol_type = other DNA
agattctataaactgtgcggtccttnnnnnngcggcatgatctaccttaaagcttgggtacggcgctatcatgtactcatg

SEQ ID NO: 193 - DNA, 81 bp, synthetic construct
  misc_feature 1..81: note = Artificial sequence
  misc_feature 1..81: note = 1OS-1-Oligo-66; Biotin-C6 in 5'; n: any of A, T, G, C independently
  source 1..81: mol_type = other DNA
agattctataaactgtgcggtccttnnnnnnccggcgcagaagtttgaacgaaaagggtacggcgctatcatgtactcatg

SEQ ID NO: 194 - DNA, 81 bp, synthetic construct
  misc_feature 1..81: note = Artificial sequence
  misc_feature 1..81: note = 1OS-1-Oligo-67; Biotin-C6 in 5'; n: any of A, T, G, C independently
  source 1..81: mol_type = other DNA
agattctataaactgtgcggtccttnnnnnnatgcactattttacgtatcccgtgcggtacggcgctatcatgtactcatg

SEQ ID NO: 195 - DNA, 81 bp, synthetic construct
  misc_feature 1..81: note = Artificial sequence
  misc_feature 1..81: note = 1OS-1-Oligo-68; Biotin-C6 in 5'; n: any of A, T, G, C independently
  source 1..81: mol_type = other DNA
agattctataaactgtgcggtccttnnnnnngatagggtgactgctttcgcgtacaggtacggcgctatcatgtactcatg

SEQ ID NO: 196 - DNA, 81 bp, synthetic construct
  misc_feature 1..81: note = Artificial sequence
  misc_feature 1..81: note = 1OS-1-Oligo-69; Biotin-C6 in 5'; n: any of A, T, G, C independently
  source 1..81: mol_type = other DNA
agattctataaactgtgcggtccttnnnnnntatctggtagacatctcggcacagaggtacggcgctatcatgtactcatg

SEQ ID NO: 197 - DNA, 81 bp, synthetic construct
  misc_feature 1..81: note = Artificial sequence
  misc_feature 1..81: note = 1OS-1-Oligo-70; Biotin-C6 in 5'; n: any of A, T, G, C independently
  source 1..81: mol_type = other DNA
agattctataaactgtgcggtccttnnnnnntcggggtgcaataatcactagtgctggtacggcgctatcatgtactcatg

SEQ ID NO: 198 - DNA, 81 bp, synthetic construct
  misc_feature 1..81: note = Artificial sequence
  misc_feature 1..81: note = 1OS-1-Oligo-71; Biotin-C6 in 5'; n: any of A, T, G, C independently
  source 1..81: mol_type = other DNA
agattctataaactgtgcggtccttnnnnnntagttctggctatacacacttcgggggtacggcgctatcatgtactcatg

SEQ ID NO: 199 - DNA, 81 bp, synthetic construct
  misc_feature 1..81: note = Artificial sequence
  misc_feature 1..81: note = 1OS-1-Oligo-72; Biotin-C6 in 5'; n: any of A, T, G, C independently
  source 1..81: mol_type = other DNA
agattctataaactgtgcggtccttnnnnnngcatagagttacccgatggattcgaggtacggcgctatcatgtactcatg

SEQ ID NO: 200 - DNA, 81 bp, synthetic construct
  misc_feature 1..81: note = Artificial sequence
  misc_feature 1..81: note = 1OS-1-Oligo-73; Biotin-C6 in 5'; n: any of A, T, G, C independently
  source 1..81: mol_type = other DNA
agattctataaactgtgcggtccttnnnnnngttcatggtacaggcttctttacggggtacggcgctatcatgtactcatg

SEQ ID NO: 201 - DNA, 81 bp, synthetic construct
  misc_feature 1..81: note = Artificial sequence
  misc_feature 1..81: note = 1OS-1-Oligo-74; Biotin-C6 in 5'; n: any of A, T, G, C independently
  source 1..81: mol_type = other DNA
agattctataaactgtgcggtccttnnnnnncgatctcgggcctgggttttgagtaggtacggcgctatcatgtactcatg

SEQ ID NO: 202 - DNA, 81 bp, synthetic construct
  misc_feature 1..81: note = Artificial sequence
  misc_feature 1..81: note = 1OS-1-Oligo-75; Biotin-C6 in 5'; n: any of A, T, G, C independently
  source 1..81: mol_type = other DNA
agattctataaactgtgcggtccttnnnnnnattattcgtgacccaactcatcaggggtacggcgctatcatgtactcatg

SEQ ID NO: 203 - DNA, 81 bp, synthetic construct
  misc_feature 1..81: note = Artificial sequence
  misc_feature 1..81: note = 1OS-1-Oligo-76; Biotin-C6 in 5'; n: any of A, T, G, C independently
  source 1..81: mol_type = other DNA
agattctataaactgtgcggtccttnnnnnnctgaatggtgaataatgcgttcgccggtacggcgctatcatgtactcatg

SEQ ID NO: 204 - DNA, 81 bp, synthetic construct
  misc_feature 1..81: note = Artificial sequence
  misc_feature 1..81: note = 1OS-1-Oligo-77; Biotin-C6 in 5'; n: any of A, T, G, C independently
  source 1..81: mol_type = other DNA
agattctataaactgtgcggtccttnnnnnngctattagttgctaccccaagaatcggtacggcgctatcatgtactcatg

SEQ ID NO: 205 - DNA, 81 bp, synthetic construct
  misc_feature 1..81: note = Artificial sequence
  misc_feature 1..81: note = 1OS-1-Oligo-78; Biotin-C6 in 5'; n: any of A, T, G, C independently
  source 1..81: mol_type = other DNA
agattctataaactgtgcggtccttnnnnnnagaaagtcttggatacacggccgggggtacggcgctatcatgtactcatg

SEQ ID NO: 206 - DNA, 81 bp, synthetic construct
  misc_feature 1..81: note = Artificial sequence
  misc_feature 1..81: note = 1OS-1-Oligo-79; Biotin-C6 in 5'; n: any of A, T, G, C independently
  source 1..81: mol_type = other DNA
agattctataaactgtgcggtccttnnnnnngtgtgttcctatgcacaatttcataggtacggcgctatcatgtactcatg

SEQ ID NO: 207 - DNA, 81 bp, synthetic construct
  misc_feature 1..81: note = Artificial sequence
  misc_feature 1..81: note = 1OS-1-Oligo-80; Biotin-C6 in 5'; n: any of A, T, G, C independently
  source 1..81: mol_type = other DNA
agattctataaactgtgcggtccttnnnnnntacatggtaggggtctccgaaccgtggtacggcgctatcatgtactcatg

SEQ ID NO: 208 - DNA, 81 bp, synthetic construct
  misc_feature 1..81: note = Artificial sequence
  misc_feature 1..81: note = 1OS-1-Oligo-81; Biotin-C6 in 5'; n: any of A, T, G, C independently
  source 1..81: mol_type = other DNA
agattctataaactgtgcggtccttnnnnnntagggataactttcctcccacttggggtacggcgctatcatgtactcatg

SEQ ID NO: 209 - DNA, 81 bp, synthetic construct
  misc_feature 1..81: note = Artificial sequence
  misc_feature 1..81: note = 1OS-1-Oligo-82; Biotin-C6 in 5'; n: any of A, T, G, C independently
  source 1..81: mol_type = other DNA
agattctataaactgtgcggtccttnnnnnntctggtgtctcacccatgggatgtcggtacggcgctatcatgtactcatg

SEQ ID NO: 210 - DNA, 81 bp, synthetic construct
  misc_feature 1..81: note = Artificial sequence
  misc_feature 1..81: note = 1OS-1-Oligo-83; Biotin-C6 in 5'; n: any of A, T, G, C independently
  source 1..81: mol_type = other DNA
agattctataaactgtgcggtccttnnnnnntaacgattttctcgcgggagtttcgggtacggcgctatcatgtactcatg

SEQ ID NO: 211 - DNA, 81 bp, synthetic construct
  misc_feature 1..81: note = Artificial sequence
  misc_feature 1..81: note = 1OS-1-Oligo-84; Biotin-C6 in 5'; n: any of A, T, G, C independently
  source 1..81: mol_type = other DNA
agattctataaactgtgcggtccttnnnnnncgagcctggttagcgcctacaagagggtacggcgctatcatgtactcatg

SEQ ID NO: 212 - DNA, 81 bp, synthetic construct
  misc_feature 1..81: note = Artificial sequence
  misc_feature 1..81: note = 1OS-1-Oligo-85; Biotin-C6 in 5'; n: any of A, T, G, C independently
  source 1..81: mol_type = other DNA
agattctataaactgtgcggtccttnnnnnncgtagtaagatatgtagtccacgtcggtacggcgctatcatgtactcatg

SEQ ID NO: 213 - DNA, 81 bp, synthetic construct
  misc_feature 1..81: note = Artificial sequence
  misc_feature 1..81: note = 1OS-1-Oligo-86; Biotin-C6 in 5'; n: any of A, T, G, C independently
  source 1..81: mol_type = other DNA
agattctataaactgtgcggtccttnnnnnntgttagttgccccatatctttacgcggtacggcgctatcatgtactcatg

SEQ ID NO: 214 - DNA, 81 bp, synthetic construct
  misc_feature 1..81: note = Artificial sequence
  misc_feature 1..81: note = 1OS-1-Oligo-87; Biotin-C6 in 5'; n: any of A, T, G, C independently
  source 1..81: mol_type = other DNA
agattctataaactgtgcggtccttnnnnnngctggattgtgattgtccggatccgggtacggcgctatcatgtactcatg

SEQ ID NO: 215 - DNA, 81 bp, synthetic construct
  misc_feature 1..81: note = Artificial sequence
  misc_feature 1..81: note = 1OS-1-Oligo-88; Biotin-C6 in 5'; n: any of A, T, G, C independently
  source 1..81: mol_type = other DNA
agattctataaactgtgcggtccttnnnnnngggaggactgcggttcagcttacaaggtacggcgctatcatgtactcatg

SEQ ID NO: 216 - DNA, 81 bp, synthetic construct
  misc_feature 1..81: note = Artificial sequence
  misc_feature 1..81: note = 1OS-1-Oligo-89; Biotin-C6 in 5'; n: any of A, T, G, C independently
  source 1..81: mol_type = other DNA
agattctataaactgtgcggtccttnnnnnngcgtaggtctagttcagattctataggtacggcgctatcatgtactcatg

SEQ ID NO: 217 - DNA, 81 bp, synthetic construct
  misc_feature 1..81: note = Artificial sequence
  misc_feature 1..81: note = 1OS-1-Oligo-90; Biotin-C6 in 5'; n: any of A, T, G, C independently
  source 1..81: mol_type = other DNA
agattctataaactgtgcggtccttnnnnnngtctacgtggttctataccattcggggtacggcgctatcatgtactcatg

SEQ ID NO: 218 - DNA, 81 bp, synthetic construct
  misc_feature 1..81: note = Artificial sequence
  misc_feature 1..81: note = 1OS-1-Oligo-91; Biotin-C6 in 5'; n: any of A, T, G, C independently
  source 1..81: mol_type = other DNA
agattctataaactgtgcggtccttnnnnnnaggctttactacaatgcgtgggctcggtacggcgctatcatgtactcatg

SEQ ID NO: 219 - DNA, 81 bp, synthetic construct
  misc_feature 1..81: note = Artificial sequence
  misc_feature 1..81: note = 1OS-1-Oligo-92; Biotin-C6 in 5'; n: any of A, T, G, C independently
  source 1..81: mol_type = other DNA
agattctataaactgtgcggtccttnnnnnnagcttgctgtatgggtcatgttcctggtacggcgctatcatgtactcatg

SEQ ID NO: 220 - DNA, 81 bp, synthetic construct
  misc_feature 1..81: note = Artificial sequence
  misc_feature 1..81: note = 1OS-1-Oligo-93; Biotin-C6 in 5'; n: any of A, T, G, C independently
  source 1..81: mol_type = other DNA
agattctataaactgtgcggtccttnnnnnntgctctaaagacgcgaggactacctggtacggcgctatcatgtactcatg

SEQ ID NO: 221 - DNA, 81 bp, synthetic construct
  misc_feature 1..81: note = Artificial sequence
  misc_feature 1..81: note = 1OS-1-Oligo-94; Biotin-C6 in 5'; n: any of A, T, G, C independently
  source 1..81: mol_type = other DNA
agattctataaactgtgcggtccttnnnnnntgtacatgtcatactcaaggctttaggtacggcgctatcatgtactcatg

SEQ ID NO: 222 - DNA, 81 bp, synthetic construct
  misc_feature 1..81: note = Artificial sequence
  misc_feature 1..81: note = 1OS-1-Oligo-95; Biotin-C6 in 5'; n: any of A, T, G, C independently
  source 1..81: mol_type = other DNA
agattctataaactgtgcggtccttnnnnnnttgacatgtacgccatttgggtcgcggtacggcgctatcatgtactcatg

SEQ ID NO: 223 - DNA, 81 bp, synthetic construct
  misc_feature 1..81: note = Artificial sequence
  misc_feature 1..81: note = 1OS-1-Oligo-96; Biotin-C6 in 5'; n: any of A, T, G, C independently
  source 1..81: mol_type = other DNA
agattctataaactgtgcggtccttnnnnnngcaattcagtacgatcgtgtagcggggtacggcgctatcatgtactcatg

SEQ ID NO: 224 - DNA, 81 bp, synthetic construct
  misc_feature 1..81: note = Artificial sequence
  misc_feature 1..81: note = 1OS-1-Oligo-97; Biotin-C6 in 5'; n: any of A, T, G, C independently
  source 1..81: mol_type = other DNA
agattctataaactgtgcggtccttnnnnnncgctgtccaaaggttcttcgtaacgggtacggcgctatcatgtactcatg

SEQ ID NO: 225 - DNA, 81 bp, synthetic construct
  misc_feature 1..81: note = Artificial sequence
  misc_feature 1..81: note = 1OS-1-Oligo-98; Biotin-C6 in 5'; n: any of A, T, G, C independently
  source 1..81: mol_type = other DNA
agattctataaactgtgcggtccttnnnnnnttagacgagcaggtttcttgcctatggtacggcgctatcatgtactcatg

SEQ ID NO: 226 - DNA, 81 bp, synthetic construct
  misc_feature 1..81: note = Artificial sequence
  misc_feature 1..81: note = 1OS-1-Oligo-99; Biotin-C6 in 5'; n: any of A, T, G, C independently
  source 1..81: mol_type = other DNA
agattctataaactgtgcggtccttnnnnnntcgtttggagccgttcacacatgaaggtacggcgctatcatgtactcatg

SEQ ID NO: 227 - DNA, 81 bp, synthetic construct
  misc_feature 1..81: note = Artificial sequence
  misc_feature 1..81: note = 1OS-1-Oligo-100; Biotin-C6 in 5'; n: any of A, T, G, C independently
  source 1..81: mol_type = other DNA
agattctataaactgtgcggtccttnnnnnnctgatcaacttgcgcccagcgttatggtacggcgctatcatgtactcatg

SEQ ID NO: 228 - DNA, 81 bp, synthetic construct
  misc_feature 1..81: note = Artificial sequence
  misc_feature 1..81: note = 1OS-1-Oligo-101; Biotin-C6 in 5'; n: any of A, T, G, C independently
  source 1..81: mol_type = other DNA
agattctataaactgtgcggtccttnnnnnngacgatgttgcctgttttgatacgaggtacggcgctatcatgtactcatg

SEQ ID NO: 229 - DNA, 81 bp, synthetic construct
  misc_feature 1..81: note = Artificial sequence
  misc_feature 1..81: note = 1OS-1-Oligo-102; Biotin-C6 in 5'; n: any of A, T, G, C independently
  source 1..81: mol_type = other DNA
agattctataaactgtgcggtccttnnnnnngggtagtcgtgaggtgaactcttccggtacggcgctatcatgtactcatg

SEQ ID NO: 230 - DNA, 81 bp, synthetic construct
  misc_feature 1..81: note = Artificial sequence
  misc_feature 1..81: note = 1OS-1-Oligo-102; Biotin-C6 in 5'; n: any of A, T, G, C independently
  source 1..81: mol_type = other DNA
agattctataaactgtgcggtccttnnnnnnagccattttacgattctattcgatgggtacggcgctatcatgtactcatg

SEQ ID NO: 231 - DNA, 81 bp, synthetic construct
  misc_feature 1..81: note = Artificial sequence
  misc_feature 1..81: note = 1OS-1-Oligo-104; Biotin-C6 in 5'; n: any of A, T, G, C independently
  source 1..81: mol_type = other DNA
agattctataaactgtgcggtccttnnnnnngtggtttatataatcccacctcctaggtacggcgctatcatgtactcatg

SEQ ID NO: 232 - DNA, 81 bp, synthetic construct
  misc_feature 1..81: note = Artificial sequence
  misc_feature 1..81: note = 1OS-1-Oligo-105; Biotin-C6 in 5'; n: any of A, T, G, C independently
  source 1..81: mol_type = other DNA
agattctataaactgtgcggtccttnnnnnngcgaagaacatcccggcatttcatgggtacggcgctatcatgtactcatg

SEQ ID NO: 233 - DNA, 81 bp, synthetic construct
  misc_feature 1..81: note = Artificial sequence
  misc_feature 1..81: note = 1OS-1-Oligo-106; Biotin-C6 in 5'; n: any of A, T, G, C independently
  source 1..81: mol_type = other DNA
agattctataaactgtgcggtccttnnnnnngctgggacaatgccgaaaactcttcggtacggcgctatcatgtactcatg

SEQ ID NO: 234 - DNA, 81 bp, synthetic construct
  misc_feature 1..81: note = Artificial sequence
  misc_feature 1..81: note = 1OS-1-Oligo-107; Biotin-C6 in 5'; n: any of A, T, G, C independently
  source 1..81: mol_type = other DNA
agattctataaactgtgcggtccttnnnnnnattccgtaccaacccgcgtcttagaggtacggcgctatcatgtactcatg

SEQ ID NO: 235 - DNA, 81 bp, synthetic construct
  misc_feature 1..81: note = Artificial sequence
  misc_feature 1..81: note = 1OS-1-Oligo-108; Biotin-C6 in 5'; n: any of A, T, G, C independently
  source 1..81: mol_type = other DNA
agattctataaactgtgcggtccttnnnnnnctgcaggaggctctaatgcactcaaggtacggcgctatcatgtactcatg

SEQ ID NO: 236 - DNA, 81 bp, synthetic construct
  misc_feature 1..81: note = Artificial sequence
  misc_feature 1..81: note = 1OS-1-Oligo-109; Biotin-C6 in 5'; n: any of A, T, G, C independently
  source 1..81: mol_type = other DNA
agattctataaactgtgcggtccttnnnnnngcgttcagcattcattacgtctcacggtacggcgctatcatgtactcatg

SEQ ID NO: 237 - DNA, 81 bp, synthetic construct
  misc_feature 1..81: note = Artificial sequence
  misc_feature 1..81: note = 1OS-1-Oligo-110; Biotin-C6 in 5'; n: any of A, T, G, C independently
  source 1..81: mol_type = other DNA
agattctataaactgtgcggtccttnnnnnngctgaggaagcccaatgttcagtacggtacggcgctatcatgtactcatg

SEQ ID NO: 238 - DNA, 81 bp, synthetic construct
  misc_feature 1..81: note = Artificial sequence
  misc_feature 1..81: note = 1OS-1-Oligo-111; Biotin-C6 in 5'; n: any of A, T, G, C independently
  source 1..81: mol_type = other DNA
agattctataaactgtgcggtccttnnnnnngtaaccttagcacgccggagtggagggtacggcgctatcatgtactcatg

SEQ ID NO: 239 - DNA, 81 bp, synthetic construct
  misc_feature 1..81: note = Artificial sequence
  misc_feature 1..81: note = 1OS-1-Oligo-112; Biotin-C6 in 5'; n: any of A, T, G, C independently
  source 1..81: mol_type = other DNA
agattctataaactgtgcggtccttnnnnnngcgattagttctgttgctaaaccagggtacggcgctatcatgtactcatg

SEQ ID NO: 240 - DNA, 81 bp, synthetic construct
  misc_feature 1..81: note = Artificial sequence
  misc_feature 1..81: note = 1OS-1-Oligo-113; Biotin-C6 in 5'; n: any of A, T, G, C independently
  source 1..81: mol_type = other DNA
agattctataaactgtgcggtccttnnnnnnccttatgagagctcgttgttcggtgggtacggcgctatcatgtactcatg

SEQ ID NO: 241 - DNA, 81 bp, synthetic construct
  misc_feature 1..81: note = Artificial sequence
  misc_feature 1..81: note = 1OS-1-Oligo-114; Biotin-C6 in 5'; n: any of A, T, G, C independently
  source 1..81: mol_type = other DNA
agattctataaactgtgcggtccttnnnnnncttaaaggtgattcacacgtgtgccggtacggcgctatcatgtactcatg

SEQ ID NO: 242 - DNA, 81 bp, synthetic construct
  misc_feature 1..81: note = Artificial sequence
  misc_feature 1..81: note = 1OS-1-Oligo-115; Biotin-C6 in 5'; n: any of A, T, G, C independently
  source 1..81: mol_type = other DNA
agattctataaactgtgcggtccttnnnnnnttactgagtaacgttctaccccgaaggtacggcgctatcatgtactcatg

SEQ ID NO: 243 - DNA, 81 bp, synthetic construct
  misc_feature 1..81: note = Artificial sequence
  misc_feature 1..81: note = 1OS-1-Oligo-116; Biotin-C6 in 5'; n: any of A, T, G, C independently
  source 1..81: mol_type = other DNA
agattctataaactgtgcggtccttnnnnnnatacttattccgctcattgcacaggggtacggcgctatcatgtactcatg

SEQ ID NO: 244 - DNA, 81 bp, synthetic construct
  misc_feature 1..81: note = Artificial sequence
  misc_feature 1..81: note = 1OS-1-Oligo-117; Biotin-C6 in 5'; n: any of A, T, G, C independently
  source 1..81: mol_type = other DNA
agattctataaactgtgcggtccttnnnnnntgaaaccaatttcacctcagcggcgggtacggcgctatcatgtactcatg

SEQ ID NO: 245 - DNA, 81 bp, synthetic construct
  misc_feature 1..81: note = Artificial sequence
  misc_feature 1..81: note = 1OS-1-Oligo-118; Biotin-C6 in 5'; n: any of A, T, G, C independently
  source 1..81: mol_type = other DNA
agattctataaactgtgcggtccttnnnnnngcgatcggtaggtaccttttcagtaggtacggcgctatcatgtactcatg

SEQ ID NO: 246 - DNA, 58 bp, synthetic construct
  misc_feature 1..58: note = Artificial sequence
  misc_feature 1..58: note = A-Key 2OS-F1-16
  source 1..58: mol_type = other DNA
ccatctcatccctgcgtgtctccgactcagtgttgcgttagaagttccagccagcgtc

SEQ ID NO: 247 - DNA, 58 bp, synthetic construct
  misc_feature 1..58: note = Artificial sequence
  misc_feature 1..58: note = A-Key 2OS-F1-17
  source 1..58: mol_type = other DNA
ccatctcatccctgcgtgtctccgactcagtgcgagcgaggaagttccagccagcgtc

SEQ ID NO: 248 - DNA, 58 bp, synthetic construct
  misc_feature 1..58: note = Artificial sequence
  misc_feature 1..58: note = A-Key 2OS-F1-18
  source 1..58: mol_type = other DNA
ccatctcatccctgcgtgtctccgactcagtgcgactctggaagttccagccagcgtc

SEQ ID NO: 249 - DNA, 58 bp, synthetic construct
  misc_feature 1..58: note = Artificial sequence
  misc_feature 1..58: note = A-Key 2OS-F1-19
  source 1..58: mol_type = other DNA
ccatctcatccctgcgtgtctccgactcagtgatccgtccgaagttccagccagcgtc

SEQ ID NO: 250 - DNA, 58 bp, synthetic construct
  misc_feature 1..58: note = Artificial sequence
  misc_feature 1..58: note = A-Key 2OS-F1-20
  source 1..58: mol_type = other DNA
ccatctcatccctgcgtgtctccgactcagtgttaaacgagaagttccagccagcgtc

SEQ ID NO: 251 - DNA, 58 bp, synthetic construct
  misc_feature 1..58: note = Artificial sequence
  misc_feature 1..58: note = A-Key 2OS-F1-21
  source 1..58: mol_type = other DNA
ccatctcatccctgcgtgtctccgactcagtgtagcttttgaagttccagccagcgtc

SEQ ID NO: 252 - DNA, 58 bp, synthetic construct
  misc_feature 1..58: note = Artificial sequence
  misc_feature 1..58: note = A-Key 2OS-F1-22
  source 1..58: mol_type = other DNA
ccatctcatccctgcgtgtctccgactcagtgcacatgtagaagttccagccagcgtc

SEQ ID NO: 253 - DNA, 58 bp, synthetic construct
  misc_feature 1..58: note = Artificial sequence
  misc_feature 1..58: note = A-Key 2OS-F1-23
  source 1..58: mol_type = other DNA
ccatctcatccctgcgtgtctccgactcagtggatagccagaagttccagccagcgtc

SEQ ID NO: 254 - DNA, 58 bp, synthetic construct
  misc_feature 1..58: note = Artificial sequence
  misc_feature 1..58: note = A-Key 2OS-F1-24
  source 1..58: mol_type = other DNA
ccatctcatccctgcgtgtctccgactcagtgacctgttagaagttccagccagcgtc

SEQ ID NO: 255 - DNA, 58 bp, synthetic construct
  misc_feature 1..58: note = Artificial sequence
  misc_feature 1..58: note = A-Key 2OS-F1-25
  source 1..58: mol_type = other DNA
ccatctcatccctgcgtgtctccgactcagtgtgcgaattgaagttccagccagcgtc

SEQ ID NO: 256 - DNA, 58 bp, synthetic construct
  misc_feature 1..58: note = Artificial sequence
  misc_feature 1..58: note = A-Key 2OS-F1-26
  source 1..58: mol_type = other DNA
ccatctcatccctgcgtgtctccgactcagtggtacatttgaagttccagccagcgtc

SEQ ID NO: 257 - DNA, 58 bp, synthetic construct
  misc_feature 1..58: note = Artificial sequence
  misc_feature 1..58: note = A-Key 2OS-F1-27
  source 1..58: mol_type = other DNA
ccatctcatccctgcgtgtctccgactcagtgctattgcagaagttccagccagcgtc

SEQ ID NO: 258 - DNA, 58 bp, synthetic construct
  misc_feature 1..58: note = Artificial sequence
  misc_feature 1..58: note = A-Key 2OS-F1-28
  source 1..58: mol_type = other DNA
ccatctcatccctgcgtgtctccgactcagtgacgatacagaagttccagccagcgtc

SEQ ID NO: 259 - DNA, 58 bp, synthetic construct
  misc_feature 1..58: note = Artificial sequence
  misc_feature 1..58: note = A-Key 2OS-F1-29
  source 1..58: mol_type = other DNA
ccatctcatccctgcgtgtctccgactcagtgcttagcgcgaagttccagccagcgtc

SEQ ID NO: 260 - DNA, 58 bp, synthetic construct
  misc_feature 1..58: note = Artificial sequence
  misc_feature 1..58: note = A-Key 2OS-F1-30
  source 1..58: mol_type = other DNA
ccatctcatccctgcgtgtctccgactcagtgcggaaaccgaagttccagccagcgtc

SEQ ID NO: 261 - DNA, 58 bp, synthetic construct
  misc_feature 1..58: note = Artificial sequence
  misc_feature 1..58: note = A-Key 2OS-F1-31
  source 1..58: mol_type = other DNA
ccatctcatccctgcgtgtctccgactcagtggatgttgggaagttccagccagcgtc

SEQ ID NO: 262 - DNA, 58 bp, synthetic construct
  misc_feature 1..58: note = Artificial sequence
  misc_feature 1..58: note = A-Key 2OS-F1-32
  source 1..58: mol_type = other DNA
ccatctcatccctgcgtgtctccgactcagtgatcggcgtgaagttccagccagcgtc

SEQ ID NO: 263 - DNA, 58 bp, synthetic construct
  misc_feature 1..58: note = Artificial sequence
  misc_feature 1..58: note = A-Key 2OS-F1-33
  source 1..58: mol_type = other DNA
ccatctcatccctgcgtgtctccgactcagtgtagtacgagaagttccagccagcgtc

SEQ ID NO: 264 - DNA, 58 bp, synthetic construct
  misc_feature 1..58: note = Artificial sequence
  misc_feature 1..58: note = A-Key 2OS-F1-34
  source 1..58: mol_type = other DNA
ccatctcatccctgcgtgtctccgactcagtggacgtgatgaagttccagccagcgtc

SEQ ID NO: 265 - DNA, 58 bp, synthetic construct
  misc_feature 1..58: note = Artificial sequence
  misc_feature 1..58: note = A-Key 2OS-F1-35
  source 1..58: mol_type = other DNA
ccatctcatccctgcgtgtctccgactcagtgtgagccaagaagttccagccagcgtc

SEQ ID NO: 266 - DNA, 58 bp, synthetic construct
  misc_feature 1..58: note = Artificial sequence
  misc_feature 1..58: note = A-Key 2OS-F1-36
  source 1..58: mol_type = other DNA
ccatctcatccctgcgtgtctccgactcagtgcctcgcaggaagttccagccagcgtc

SEQ ID NO: 267 - DNA, 58 bp, synthetic construct
  misc_feature 1..58: note = Artificial sequence
  misc_feature 1..58: note = A-Key 2OS-F1-37
  source 1..58: mol_type = other DNA
ccatctcatccctgcgtgtctccgactcagtgagatccaggaagttccagccagcgtc

SEQ ID NO: 268 - DNA, 58 bp, synthetic construct
  misc_feature 1..58: note = Artificial sequence
  misc_feature 1..58: note = A-Key 2OS-F1-38
  source 1..58: mol_type = other DNA
ccatctcatccctgcgtgtctccgactcagtgttggctgagaagttccagccagcgtc

SEQ ID NO: 269 - DNA, 58 bp, synthetic construct
  misc_feature 1..58: note = Artificial sequence
  misc_feature 1..58: note = A-Key 2OS-F1-39
  source 1..58: mol_type = other DNA
ccatctcatccctgcgtgtctccgactcagtggaccgctagaagttccagccagcgtc

SEQ ID NO: 270 - DNA, 58 bp, synthetic construct
  misc_feature 1..58: note = Artificial sequence
  misc_feature 1..58: note = A-Key 2OS-F1-40
  source 1..58: mol_type = other DNA
ccatctcatccctgcgtgtctccgactcagtggagcttaagaagttccagccagcgtc

SEQ ID NO: 271 - DNA, 58 bp, synthetic construct
  misc_feature 1..58: note = Artificial sequence
  misc_feature 1..58: note = A-Key 2OS-F1-41
  source 1..58: mol_type = other DNA
ccatctcatccctgcgtgtctccgactcagtgggactggtgaagttccagccagcgtc

SEQ ID NO: 272 - DNA, 58 bp, synthetic construct
  misc_feature 1..58: note = Artificial sequence
  misc_feature 1..58: note = A-Key 2OS-F1-42
  source 1..58: mol_type = other DNA
ccatctcatccctgcgtgtctccgactcagtgtgggagtcgaagttccagccagcgtc

SEQ ID NO: 273 - DNA, 58 bp, synthetic construct
  misc_feature 1..58: note = Artificial sequence
  misc_feature 1..58: note = A-Key 2OS-F1-43
  source 1..58: mol_type = other DNA
ccatctcatccctgcgtgtctccgactcagtggcgatggcgaagttccagccagcgtc

SEQ ID NO: 274 - DNA, 58 bp, synthetic construct
  misc_feature 1..58: note = Artificial sequence
  misc_feature 1..58: note = A-Key 2OS-F1-44
  source 1..58: mol_type = other DNA
ccatctcatccctgcgtgtctccgactcagtgacttggttgaagttccagccagcgtc

SEQ ID NO: 275 - DNA, 58 bp, synthetic construct
  misc_feature 1..58: note = Artificial sequence
  misc_feature 1..58: note = A-Key 2OS-F1-45
  source 1..58: mol_type = other DNA
ccatctcatccctgcgtgtctccgactcagtgatactcatgaagttccagccagcgtc

SEQ ID NO: 276 - DNA, 58 bp, synthetic construct
  misc_feature 1..58: note = Artificial sequence
  misc_feature 1..58: note = A-Key 2OS-F1-46
  source 1..58: mol_type = other DNA
ccatctcatccctgcgtgtctccgactcagtgtagtgtccgaagttccagccagcgtc

SEQ ID NO: 277 - DNA, 58 bp, synthetic construct
  misc_feature 1..58: note = Artificial sequence
  misc_feature 1..58: note = A-Key 2OS-F1-47
  source 1..58: mol_type = other DNA
ccatctcatccctgcgtgtctccgactcagtggcatataagaagttccagccagcgtc

SEQ ID NO: 278 - DNA, 58 bp, synthetic construct
  misc_feature 1..58: note = Artificial sequence
  misc_feature 1..58: note = A-Key 2OS-F1-48
  source 1..58: mol_type = other DNA
ccatctcatccctgcgtgtctccgactcagtgggcgattggaagttccagccagcgtc

SEQ ID NO: 279 - DNA, 58 bp, synthetic construct
  misc_feature 1..58: note = Artificial sequence
  misc_feature 1..58: note = A-Key 2OS-F1-49
  source 1..58: mol_type = other DNA
ccatctcatccctgcgtgtctccgactcagtggggctgtagaagttccagccagcgtc

SEQ ID NO: 280 - DNA, 58 bp, synthetic construct
  misc_feature 1..58: note = Artificial sequence
  misc_feature 1..58: note = A-Key 2OS-F1-50
  source 1..58: mol_type = other DNA
ccatctcatccctgcgtgtctccgactcagtgcgctatttgaagttccagccagcgtc

SEQ ID NO: 281 - DNA, 58 bp, synthetic construct
  misc_feature 1..58: note = Artificial sequence
  misc_feature 1..58: note = A-Key 2OS-F1-51
  source 1..58: mol_type = other DNA
ccatctcatccctgcgtgtctccgactcagtggtactgcagaagttccagccagcgtc

SEQ ID NO: 282 - DNA, 58 bp, synthetic construct
  misc_feature 1..58: note = Artificial sequence
  misc_feature 1..58: note = A-Key 2OS-F1-52
  source 1..58: mol_type = other DNA
ccatctcatccctgcgtgtctccgactcagtgtgtctatggaagttccagccagcgtc

SEQ ID NO: 283 - DNA, 58 bp, synthetic construct
  misc_feature 1..58: note = Artificial sequence
  misc_feature 1..58: note = A-Key 2OS-F1-53
  source 1..58: mol_type = other DNA
ccatctcatccctgcgtgtctccgactcagtgcgaatcacgaagttccagccagcgtc

SEQ ID NO: 284 - DNA, 58 bp, synthetic construct
  misc_feature 1..58: note = Artificial sequence
  misc_feature 1..58: note = A-Key 2OS-F1-54
  source 1..58: mol_type = other DNA
ccatctcatccctgcgtgtctccgactcagtgcgtcctaagaagttccagccagcgtc

SEQ ID NO: 285 - DNA, 58 bp, synthetic construct
  misc_feature 1..58: note = Artificial sequence
  misc_feature 1..58: note = A-Key 2OS-F1-55
  source 1..58: mol_type = other DNA
ccatctcatccctgcgtgtctccgactcagtgacaaatgggaagttccagccagcgtc

SEQ ID NO: 286 - DNA, 58 bp, synthetic construct
  misc_feature 1..58: note = Artificial sequence
  misc_feature 1..58: note = A-Key 2OS-F1-56
  source 1..58: mol_type = other DNA
ccatctcatccctgcgtgtctccgactcagtgtctactttgaagttccagccagcgtc

SEQ ID NO: 287 - DNA, 58 bp, synthetic construct
  misc_feature 1..58: note = Artificial sequence
  misc_feature 1..58: note = A-Key 2OS-F1-57
  source 1..58: mol_type = other DNA
ccatctcatccctgcgtgtctccgactcagtgaattcgaggaagttccagccagcgtc

SEQ ID NO: 288 - DNA, 58 bp, synthetic construct
  misc_feature 1..58: note = Artificial sequence
  misc_feature 1..58: note = A-Key 2OS-F1-58
  source 1..58: mol_type = other DNA
ccatctcatccctgcgtgtctccgactcagtggaactcgggaagttccagccagcgtc

SEQ ID NO: 289 - DNA, 58 bp, synthetic construct
  misc_feature 1..58: note = Artificial sequence
  misc_feature 1..58: note = A-Key 2OS-F1-59
  source 1..58: mol_type = other DNA
ccatctcatccctgcgtgtctccgactcagtggcggacgcgaagttccagccagcgtc

SEQ ID NO: 290 - DNA, 58 bp, synthetic construct
  misc_feature 1..58: note = Artificial sequence
  misc_feature 1..58: note = A-Key 2OS-F1-60
  source 1..58: mol_type = other DNA
ccatctcatccctgcgtgtctccgactcagtgcttgtccagaagttccagccagcgtc

SEQ ID NO: 291 - DNA, 58 bp, synthetic construct
  misc_feature 1..58: note = Artificial sequence
  misc_feature 1..58: note = A-Key 2OS-F1-61
  source 1..58: mol_type = other DNA
ccatctcatccctgcgtgtctccgactcagtggtcgcggtgaagttccagccagcgtc

SEQ ID NO: 292 - DNA, 58 bp, synthetic construct
  misc_feature 1..58: note = Artificial sequence
  misc_feature 1..58: note = A-Key 2OS-F1-62
  source 1..58: mol_type = other DNA
ccatctcatccctgcgtgtctccgactcagtgcaggtcgtgaagttccagccagcgtc

SEQ ID NO: 293 - DNA, 58 bp, synthetic construct
  misc_feature 1..58: note = Artificial sequence
  misc_feature 1..58: note = A-Key 2OS-F1-63
  source 1..58: mol_type = other DNA
ccatctcatccctgcgtgtctccgactcagtgtctcatccgaagttccagccagcgtc

SEQ ID NO: 294 - DNA, 58 bp, synthetic construct
  misc_feature 1..58: note = Artificial sequence
  misc_feature 1..58: note = A-Key 2OS-F1-64
  source 1..58: mol_type = other DNA
ccatctcatccctgcgtgtctccgactcagtggcttcgtggaagttccagccagcgtc

SEQ ID NO: 295 - DNA, 58 bp, synthetic construct
  misc_feature 1..58: note = Artificial sequence
  misc_feature 1..58: note = A-Key 2OS-F1-65
  source 1..58: mol_type = other DNA
ccatctcatccctgcgtgtctccgactcagtgcgtgataagaagttccagccagcgtc

SEQ ID NO: 296 - DNA, 58 bp, synthetic construct
  misc_feature 1..58: note = Artificial sequence
  misc_feature 1..58: note = A-Key 2OS-F1-66
  source 1..58: mol_type = other DNA
ccatctcatccctgcgtgtctccgactcagtgttgctcacgaagttccagccagcgtc

SEQ ID NO: 297 - DNA, 58 bp, synthetic construct
  misc_feature 1..58: note = Artificial sequence
  misc_feature 1..58: note = A-Key 2OS-F1-67
  source 1..58: mol_type = other DNA
ccatctcatccctgcgtgtctccgactcagtgcgctctccgaagttccagccagcgtc

SEQ ID NO: 298 - DNA, 58 bp, synthetic construct
  misc_feature 1..58: note = Artificial sequence
  misc_feature 1..58: note = A-Key 2OS-F1-68
  source 1..58: mol_type = other DNA
ccatctcatccctgcgtgtctccgactcagtgattctactgaagttccagccagcgtc

SEQ ID NO: 299 - DNA, 58 bp, synthetic construct
  misc_feature 1..58: note = Artificial sequence
  misc_feature 1..58: note = A-Key 2OS-F1-69
  source 1..58: mol_type = other DNA
ccatctcatccctgcgtgtctccgactcagtgaaggcgttgaagttccagccagcgtc

SEQ ID NO: 300 - DNA, 58 bp, synthetic construct
  misc_feature 1..58: note = Artificial sequence
  misc_feature 1..58: note = A-Key 2OS-F1-70
  source 1..58: mol_type = other DNA
ccatctcatccctgcgtgtctccgactcagtggcgggattgaagttccagccagcgtc

SEQ ID NO: 301 - protein, 9 aa, synthetic construct
  REGION 1..9: note = Artificial sequence
  PEPTIDE 1..9: note = Neg Control
GPAESAAGL

SEQ ID NO: 302 - protein, 9 aa, synthetic construct
  REGION 1..9: note = Artificial sequence
  PEPTIDE 1..9: note = Neg Control
AAKGRGAAL

SEQ ID NO: 303 - protein, 9 aa, synthetic construct
  REGION 1..9: note = Artificial sequence
  PEPTIDE 1..9: note = Neg Control
AYAGSAGSI

SEQ ID NO: 304 - protein, 9 aa, synthetic construct
  REGION 1..9: note = Artificial sequence
  PEPTIDE 1..9: note = Neg Control
STEGGGLAY

SEQ ID NO: 305 - protein, 21 aa, Clostridium tetani
  PEPTIDE 1..21: note = C. tetani TT 948-968
FNNFTVSFWLRVPKVSASHLE

SEQ ID NO: 306 - protein, 9 aa, synthetic construct
  PEPTIDE 1..9: note = Dextramer 2
NLVPMVATV

SEQ ID NO: 307 - protein, 10 aa, synthetic construct
  PEPTIDE 1..10: note = CMV-derived peptide
TPRVTGGGAM

SEQ ID NO: 308 - protein, 11 aa, synthetic construct
  PEPTIDE 1..11: note = CMV pp65 YSE
YSEHPTFTSQY

SEQ ID NO: 309 - protein, 9 aa, synthetic construct
  PEPTIDE 1..9: note = CMV pp50 VTE
VTEHDTLLY

SEQ ID NO: 310 - protein, 9 aa, synthetic construct
  PEPTIDE 1..9: note = CMV IE1 VLE
VLEETSVML

SEQ ID NO: 311 - protein, 11 aa, synthetic construct
  PEPTIDE 1..11: note = CMV pp150 TTV
TTVYPPSSTAK

SEQ ID NO: 312 - protein, 10 aa, synthetic construct
  PEPTIDE 1..10: note = CMV pp150 TVY
TVYPPSSTAK

SEQ ID NO: 313 - protein, 10 aa, synthetic construct
  PEPTIDE 1..10: note = CMV pp65 RPH-L
RPHERNGFTV

SEQ ID NO: 314 - protein, 9 aa, synthetic construct
  PEPTIDE 1..9: note = CMV IE1 VLE
VLEETSVML

SEQ ID NO: 315 - protein, 10 aa, Homo sapiens
  PEPTIDE 1..10: note = 707-AP
RVAALARDAP

SEQ ID NO: 316 - protein, 9 aa, Homo sapiens
  PEPTIDE 1..9: note = ATIC (AICRT)
RLDFNLIRV

SEQ ID NO: 317 - protein, 9 aa, Homo sapiens
  PEPTIDE 1..9: note = ATIC (AICRT)
MVYDLYKTL

SEQ ID NO: 318 - protein, 9 aa, Homo sapiens
  PEPTIDE 1..9: note = BA46 (MFGE8)
NLFETPVEA

SEQ ID NO: 319 - protein, 9 aa, Homo sapiens
  PEPTIDE 1..9: note = BA46 (MFGE8)
GLQHWVPEL

SEQ ID NO: 320 - protein, 10 aa, Homo sapiens
  PEPTIDE 1..10: note = Bcl-2
PLFDFSWLSL

SEQ ID NO: 321 - protein, 10 aa, Homo sapiens
  PEPTIDE 1..10: note = Bcl-2
WLSLKTLLSL

SEQ ID NO: 322 - protein, 10 aa, Homo sapiens
  PEPTIDE 1..10: note = Bcl-xL
YLNDHLEPWI

SEQ ID NO: 323 - protein, 9 aa, Homo sapiens
  PEPTIDE 1..9: note = BING-4
CQWGRLWQL

SEQ ID NO: 324 - protein, 10 aa, Homo sapiens
  PEPTIDE 1..10: note = B-RAF
LATEKSRWSG

SEQ ID NO: 325 - protein, 8 aa, Homo sapiens
  PEPTIDE 1..8: note = cyclophilin B (Cyp-B)
VLEGMEVV

SEQ ID NO: 326 - protein, 9 aa, Homo sapiens
  PEPTIDE 1..9: note = Cadherin 3/P-cadherin
FILPVLGAV

SEQ ID NO: 327 - protein, 9 aa, Homo sapiens
  PEPTIDE 1..9: note = Cadherin 3/P-cadherin
FIIENLKAA

SEQ ID NO: 328 - protein, 9 aa, Homo sapiens
  PEPTIDE 1..9: note = CDCA1/NUF2
YMMPVNSEV

SEQ ID NO: 329 - protein, 9 aa, Homo sapiens
  PEPTIDE 1..9: note = CDCA1/NUF2
KLATAQFKI

SEQ ID NO: 330 - protein, 10 aa, Homo sapiens
  PEPTIDE 1..10: note = CDK4
ACDPHSGHFV

SEQ ID NO: 331 - protein, 9 aa, Homo sapiens
  PEPTIDE 1..9: note = CML28 (EXOSC5)
ALVDAGVPM

SEQ ID NO: 332 - protein, 9 aa, Homo sapiens
  PEPTIDE 1..9: note = COA-1 (UBXN11)
FMTRKLWDL

SEQ ID NO: 333 - protein, 9 aa, Homo sapiens
  PEPTIDE 1..9: note = COA-1 (UBXN11)
RLLASLQDL

SEQ ID NO: 334 - protein, 9 aa, Homo sapiens
  PEPTIDE 1..9: note = CPSF
KVHPVIWSL

SEQ ID NO: 335 - protein, 10 aa, Homo sapiens
  PEPTIDE 1..10: note = CPSF
LMLQNALTTM

SEQ ID NO: 336 - protein, 9 aa, Homo sapiens
  PEPTIDE 1..9: note = Cyclin I
LLDRFLATV

SEQ ID NO: 337 - protein, 9 aa, Homo sapiens
  PEPTIDE 1..9: note = cyclin B1
AGYLMELCC

SEQ ID NO: 338 - protein, 9 aa, Homo sapiens
  PEPTIDE 1..9: note = cyclin B1
AKYLMELTM

SEQ ID NO: 339 - protein, 9 aa, Homo sapiens
  PEPTIDE 1..9: note = B-RAF
LATEKSRWS

SEQ ID NO: 340 - protein, 10 aa, Homo sapiens
  PEPTIDE 1..10: note = cyclophilin B (Cyp-B)
KLKHYGPGWV

SEQ ID NO: 341 - protein, 9 aa, Homo sapiens
  PEPTIDE 1..9: note = DAM-6, -10 (MAGE-B1, -B2)
FLWGPRAYA

SEQ ID NO: 342 - protein, 9 aa, Homo sapiens
  PEPTIDE 1..9: note = EphA2
IMNDMPIYM

SEQ ID NO: 343 - protein, 9 aa, Homo sapiens
  PEPTIDE 1..9: note = EphA2
VLAGVGFFI

SEQ ID NO: 344 - protein, 9 aa, Homo sapiens
  PEPTIDE 1..9: note = EphA2
VLLLVLAGV

SEQ ID NO: 345 - protein, 9 aa, Homo sapiens
  PEPTIDE 1..9: note = EphA2
TLADFDPRV

SEQ ID NO: 346 - protein, 10 aa, Homo sapiens
  PEPTIDE 1..10: note = EZH2
FINDEIFVEL

SEQ ID NO: 347 - protein, 9 aa, Homo sapiens
  PEPTIDE 1..9: note = EZH2
FMVEDETVL

SEQ ID NO: 348 - protein, 10 aa, Homo sapiens
  PEPTIDE 1..10: note = GnTV
VLPDVFIRCV

SEQ ID NO: 349 - protein, 9 aa, Homo sapiens
  PEPTIDE 1..9: note = gp100 / Pmel17
YLEPGPVTA

SEQ ID NO: 350 - protein, 10 aa, Homo sapiens
  PEPTIDE 1..10: note = gp100 / Pmel17
LLDGTATLRL

SEQ ID NO: 351 - protein, 9 aa, Homo sapiens
  PEPTIDE 1..9: note = gp100 / Pmel17
ITDQVPFSV

SEQ ID NO: 352 - protein, 10 aa, Homo sapiens
  PEPTIDE 1..10: note = gp100 / Pmel17
VLYRYGSFSV

SEQ ID NO: 353 - protein, 9 aa, Homo sapiens
  PEPTIDE 1..9: note = gp100 / Pmel17
RLMKQDFSV

SEQ ID NO: 354 - protein, 9 aa, Homo sapiens
  PEPTIDE 1..9: note = gp100 / Pmel17
RLPRIFCSC

SEQ ID NO: 355 - protein, 10 aa, Homo sapiens
  PEPTIDE 1..10: note = gp100 / Pmel17
AMLGTHTMEV

SEQ ID NO: 356 - protein, 10 aa, Homo sapiens
  PEPTIDE 1..10: note = gp100 / Pmel17
SLADTNSLAV

SEQ ID NO: 357 - protein, 9 aa, Homo sapiens
  PEPTIDE 1..9: note = gp100 / Pmel17
KTWGQYWQV

SEQ ID NO: 358 - protein, 9 aa, Homo sapiens
  PEPTIDE 1..9: note = HERV-K-MEL
MLAVISCAV

SEQ ID NO: 359 - protein, 9 aa, Homo sapiens
  PEPTIDE 1..9: note = hsp70
LLLLDVAPL

SEQ ID NO: 360 - protein, 9 aa, Homo sapiens
  PEPTIDE 1..9: note = IDO1
ALLEIASCL

SEQ ID NO: 361 - protein, 11 aa, Homo sapiens
  PEPTIDE 1..11: note = LAGE-1
MLMAQEALAFL

SEQ ID NO: 362 - protein, 10 aa, Homo sapiens
  PEPTIDE 1..10: note = Livin (ML-IAP)
RLASFYDWLP

SEQ ID NO: 363 - protein, 9 aa, Homo sapiens
  PEPTIDE 1..9: note = Livin (ML-IAP)
SLGSPVLGL

SEQ ID NO: 364 - protein, 10 aa, Homo sapiens
  PEPTIDE 1..10: note = Livin (ML-IAP)
QLCPICRAPV

SEQ ID NO: 365 - protein, 9 aa, Homo sapiens
  PEPTIDE 1..9: note = M2BP
RIDITLSSV

SEQ ID NO: 366 - protein, 9 aa, Homo sapiens
  PEPTIDE 1..9: note = MAGE-A1
KVLEYVIKV

SEQ ID NO: 367 - protein, 9 aa, Homo sapiens
  PEPTIDE 1..9: note = GnTV
VLPDVFIRC

SEQ ID NO: 368 - protein, 9 aa, Homo sapiens
  PEPTIDE 1..9: note = gp100 / Pmel17
IMDQVPFSV

SEQ ID NO: 369 - protein, 9 aa, Homo sapiens
  PEPTIDE 1..9: note = gp100 / Pmel17
MLGTHTMEV

SEQ ID NO: 370 - protein, 9 aa, Homo sapiens
  PEPTIDE 1..9: note = hsp70
LLDVAPLSL

SEQ ID NO: 371 - protein, 9 aa, Homo sapiens
  PEPTIDE 1..9: note = MAGE-A10
GLYDGMEHL

SEQ ID NO: 372 - protein, 9 aa, Homo sapiens
  PEPTIDE 1..9: note = MAGE-A2
LVHFLLLKY

SEQ ID NO: 373 - protein, 9 aa, Homo sapiens
  PEPTIDE 1..9: note = MAGE-A2
LVQENYLEY

SEQ ID NO: 374 - protein, 10 aa, Homo sapiens
  PEPTIDE 1..10: note = MAGE-A2
YLQLVFGIEV

SEQ ID NO: 375 - protein, 9 aa, Homo sapiens
  PEPTIDE 1..9: note = MAGE-A2
KMVELVHFL

SEQ ID NO: 376 - protein, 10 aa, Homo sapiens
  PEPTIDE 1..10: note = MAGE-A3
LVFGIELMEV

SEQ ID NO: 377 - protein, 10 aa, Homo sapiens
  PEPTIDE 1..10: note = MAGE-A4
GVYDGREHTV

SEQ ID NO: 378 - protein, 9 aa, Homo sapiens
  PEPTIDE 1..9: note = MAGE-A1
YLEYRQVPV

SEQ ID NO: 379 - protein, 9 aa, Homo sapiens
  PEPTIDE 1..9: note = MAGE-A8
GLMDVQIPT

SEQ ID NO: 380 - protein, 9 aa, Homo sapiens
  PEPTIDE 1..9: note = MAGE-A8
KVAELVRFL

SEQ ID NO: 381 - protein, 9 aa, Homo sapiens
  PEPTIDE 1..9: note = MAGE-A9
ALSVMGVYV

SEQ ID NO: 382 - protein, 9 aa, Homo sapiens
  PEPTIDE 1..9: note = MAGE-C2
ALKDVEERV

SEQ ID NO: 383 - protein, 10 aa, Homo sapiens
  PEPTIDE 1..10: note = MAGE-C2
LLFGLALIEV

SEQ ID NO: 384 - protein, 9 aa, Homo sapiens
  PEPTIDE 1..9: note = MAGE-C2
VIWEVLNAV

SEQ ID NO: 385 - protein, 10 aa, Homo sapiens
  PEPTIDE 1..10: note = MAGE-C2
TLDEKVAELV

SEQ ID NO: 386 - protein, 9 aa, Homo sapiens
  PEPTIDE 1..9: note = MAGE-C2
KVLEFLAKL

SEQ ID NO: 387 - protein, 9 aa, Homo sapiens
  PEPTIDE 1..9: note = MAGE-A3
KVAELVHFL

SEQ ID NO: 388 - protein, 9 aa, Homo sapiens
  PEPTIDE 1..9: note = MC1R
TILLGIFFL

SEQ ID NO: 389 - protein, 10 aa, Homo sapiens
  PEPTIDE 1..10: note = Melan-A / MART-1
ELAGIGILTV

SEQ ID NO: 390 - protein, 9 aa, Homo sapiens
  PEPTIDE 1..9: note = Melan-A / MART-1
ILTVILGVL

SEQ ID NO: 391 - protein, 9 aa, Homo sapiens
  PEPTIDE 1..9: note = Meloe-1
TLNDECWPA

SEQ ID NO: 392 - protein, 9 aa, Homo sapiens
  PEPTIDE 1..9: note = MG50
CMHLLLEAV

SEQ ID NO: 393 - protein, 9 aa, Homo sapiens
  PEPTIDE 1..9: note = MG50
VLSVNVPDV

SEQ ID NO: 394 - protein, 9 aa, Homo sapiens
  PEPTIDE 1..9: note = NY-ESO-1 / LAGE-2
QLSLLMWIT

SEQ ID NO: 395 - protein, 11 aa, Homo sapiens
  PEPTIDE 1..11: note = NY-ESO-1 / LAGE-2
SLLMWITQCFL

SEQ ID NO: 396 - protein, 9 aa, Homo sapiens
  PEPTIDE 1..9: note = P Polypeptide
IMLCLIAAV

SEQ ID NO: 397 - protein, 9 aa, Homo sapiens
  PEPTIDE 1..9: note = p53
VVPCEPPEV

SEQ ID NO: 398 - protein, 9 aa, Homo sapiens
  PEPTIDE 1..9: note = p53
KTCPVQLWV

SEQ ID NO: 399 - protein, 9 aa, Homo sapiens
  PEPTIDE 1..9: note = p53
RMPEAAPPV

SEQ ID NO: 400 - protein, 11 aa, Homo sapiens
  PEPTIDE 1..11: note = p53
LLPENNVLSPV

SEQ ID NO: 401 - protein, 9 aa, Homo sapiens
  PEPTIDE 1..9: note = p53
KLCPVQLWV

SEQ ID NO: 402 - protein, 9 aa, Homo sapiens
  PEPTIDE 1..9: note = p53
SMPPPGTRV

SEQ ID NO: 403 - protein, 9 aa, Homo sapiens
  PEPTIDE 1..9: note = p53
LLGRNSFEV

SEQ ID NO: 404 - protein, 11 aa, Homo sapiens
  PEPTIDE 1..11: note = p53
GLAPPQHLIRV

SEQ ID NO: 405 - protein, 9 aa, Homo sapiens
  PEPTIDE 1..9: note = p53
SLPPPGTRV

SEQ ID NO: 406 - protein, 9 aa, Homo sapiens
  PEPTIDE 1..9: note = p53
YLGSYGFRL

SEQ ID NO: 407 - protein, 9 aa, Homo sapiens
  PEPTIDE 1..9: note = PGK1
IIGGGMAFT

SEQ ID NO: 408 - protein, 10 aa, Homo sapiens
  PEPTIDE 1..10: note = PRAME
ALYVDSLFFL

SEQ ID NO: 409 - protein, 9 aa, Homo sapiens
  PEPTIDE 1..9: note = PRAME
SLLQHLIGL

SEQ ID NO: 410 - protein, 10 aa, Homo sapiens
  PEPTIDE 1..10: note = SOX10
SAWISKPPGV

SEQ ID NO: 411 - protein, 10 aa, Homo sapiens
  PEPTIDE 1..10: note = PRAME
SLYSFPEPEA

SEQ ID NO: 412 - protein, 9 aa, Homo sapiens
  PEPTIDE 1..9: note = PRAME
VLDGLDVLL

SEQ ID NO: 413 - protein, 10 aa, Homo sapiens
  PEPTIDE 1..10: note = PRAME
LLLDDLLVSI

SEQ ID NO: 414 - protein, 9 aa, Homo sapiens
  PEPTIDE 1..9: note = NY-ESO-1 / LAGE-2
SLLMWITQC

SEQ ID NO: 415 - protein, 9 aa, Homo sapiens
  PEPTIDE 1..9: note = RAB38 / NY-MEL-1
VLHWDPETV

SEQ ID NO: 416 - protein, 9 aa, Homo sapiens
  PEPTIDE 1..9: note = RAGE-1
LKLSGVVRL

SEQ ID NO: 417 - protein, 10 aa, Homo sapiens
  PEPTIDE 1..10: note = RAGE-1
PLPPARNGGL

SEQ ID NO: 418 - protein, 9 aa, Homo sapiens
  PEPTIDE 1..9: note = Replication protein A
YLMDTSGKV

SEQ ID NO: 419 - protein, 9 aa, Homo sapiens
  PEPTIDE 1..9: note = SART-3
LLQAEAPRL

SEQ ID NO: 420 - protein, 9 aa, Homo sapiens
  PEPTIDE 1..9: note = SART-3
RLAEYQAYI

SEQ ID NO: 421 - protein, 9 aa, Homo sapiens
  PEPTIDE 1..9: note = secernin 1
KMDAEHPEL

SEQ ID NO: 422 - protein, 9 aa, Homo sapiens
  PEPTIDE 1..9: note = SOX10
AWISKPPGV

SEQ ID NO: 423 - protein, 9 aa, Homo sapiens
  PEPTIDE 1..9: note = SSX-2
RLQGISPKI

SEQ ID NO: 424 - protein, 9 aa, Homo sapiens
  PEPTIDE 1..9: note = SSX-2
KASEKIFYV

SEQ ID NO: 425 - protein, 9 aa, Homo sapiens
  PEPTIDE 1..9: note = STAT1-alpha/
KLQELNYNL

SEQ ID NO: 426 - protein, 9 aa, Homo sapiens
  PEPTIDE 1..9: note = STEAP1
FLYTLLREV

SEQ ID NO: 427 - protein, 9 aa, Homo sapiens
  PEPTIDE 1..9: note = STEAP1
LLLGTIHAL

SEQ ID NO: 428 - protein, 9 aa, Homo sapiens
  PEPTIDE 1..9: note = STEAP1
MIAVFLPIV

SEQ ID NO: 429 - protein, 9 aa, Homo sapiens
  PEPTIDE 1..9: note = Survivin
LMLGEFLKL

SEQ ID NO: 430 - protein, 10 aa, Homo sapiens
  PEPTIDE 1..10: note = Survivin
ELTLGEFLKL

SEQ ID NO: 431 - protein, 10 aa, Homo sapiens
  PEPTIDE 1..10: note = Survivin
TLPPAWQPFL

SEQ ID NO: 432 - protein, 9 aa, Homo sapiens
  PEPTIDE 1..9: note = TAG-1
SLGWLFLLL

SEQ ID NO: 433 - protein, 9 aa, Homo sapiens
  PEPTIDE 1..9: note = Telomerase
RLFFYRKSV

SEQ ID NO: 434 - protein, 10 aa, Homo sapiens
  PEPTIDE 1..10: note = TRP-2
VYDFFVWLHY

SEQ ID NO: 435 - protein, 9 aa, Homo sapiens
  PEPTIDE 1..9: note = NY-ESO-1 / LAGE-2
SLLMWITQA

SEQ ID NO: 436 - protein, 9 aa, Homo sapiens
  PEPTIDE 1..9: note = Telomerase
RLVDDFLLV

SEQ ID NO: 437 - protein, 9 aa, Homo sapiens
  PEPTIDE 1..9: note = Telomerase
ILAKFLHWL

SEQ ID NO: 438 - protein, 9 aa, Homo sapiens
  PEPTIDE 1..9: note = Topoisomerase II
FLYDDNQRV

SEQ ID NO: 439 - protein, 9 aa, Homo sapiens
  PEPTIDE 1..9: note = TRAG-3
ILLRDAGLV

SEQ ID NO: 440 - protein, 9 aa, Homo sapiens
  PEPTIDE 1..9: note = TRP-2
FVWLHYYSV

SEQ ID NO: 441 - protein, 9 aa, Homo sapiens
  PEPTIDE 1..9: note = TRP-2
SLDDYNHLV

SEQ ID NO: 442 - protein, 9 aa, Homo sapiens
  PEPTIDE 1..9: note = TRP-2
TLDSQVMSL

SEQ ID NO: 443 - protein, 9 aa, Homo sapiens
  PEPTIDE 1..9: note = TRP-2
SVYDFFVWL

SEQ ID NO: 444 - protein, 9 aa, Homo sapiens
  PEPTIDE 1..9: note = TRP2-6b
ATTNILEHY

SEQ ID NO: 445 - protein, 10 aa, Homo sapiens
  PEPTIDE 1..10: note = tyrosinase
CLLWSFQTSA

SEQ ID NO: 446 - protein, 9 aa, Homo sapiens
  PEPTIDE 1..9: note = tyrosinase
MLLAVLYCL

SEQ ID NO: 447 - protein, 9 aa, Homo sapiens
  PEPTIDE 1..9: note = tyrosinase
YMDGTMSQV

SEQ ID NO: 448 - protein, 9 aa, Homo sapiens
  PEPTIDE 1..9: note = XBP-1
LLSGQPASA

SEQ ID NO: 449 - protein, 9 aa, Homo sapiens
  PEPTIDE 1..9: note = MG50
LLLEAVPAV

SEQ ID NO: 450 - protein, 9 aa, Homo sapiens
  PEPTIDE 1..9: note = MG50
TLKCDCEIL

SEQ ID NO: 451 - protein, 9 aa, Homo sapiens
  PEPTIDE 1..9: note = MG50
WLPKILGEV

SEQ ID NO: 452 - protein, 9 aa, Homo sapiens
  PEPTIDE 1..9: note = MG50
RLGPTLMCL

SEQ ID NO: 453 - protein, 9 aa, Homo sapiens
  PEPTIDE 1..9: note = Meloe-2
RCPPKPPLA

SEQ ID NO: 454 - protein, 9 aa, Homo sapiens
  PEPTIDE 1..9: note = PRDX5
AMAPIKVRL

SEQ ID NO: 455 - protein, 9 aa, Homo sapiens
  PEPTIDE 1..9: note = cyclin B1
ILIDWLVQV

SEQ ID NO: 456 - protein, 10 aa, Homo sapiens
  PEPTIDE 1..10: note = Melan-A / MART-1
EAAGIGILTV

SEQ ID NO: 457 - protein, 9 aa, Homo sapiens
  PEPTIDE 1..9: note = adipophilin
SVASTITGV

SEQ ID NO: 458 - protein, 10 aa, Homo sapiens
  PEPTIDE 1..10: note = alpha-actinin-4
FIASNGVKLV

SEQ ID NO: 459 - protein, 9 aa, Homo sapiens
  PEPTIDE 1..9: note = Meloe-2
RLPPKPPLA

SEQ ID NO: 460 - protein, 9 aa, Homo sapiens
  PEPTIDE 1..9: note = CDKN1A
LMAGCIQEA

SEQ ID NO: 461 - protein, 9 aa, Homo sapiens
  PEPTIDE 1..9: note = CDKN1A
GLGLPKLYL

SEQ ID NO: 462 - protein, 9 aa, Homo sapiens
  PEPTIDE 1..9: note = CDKN1A
FAWERVRGL

SEQ ID NO: 463 - protein, 10 aa, Homo sapiens
  PEPTIDE 1..10: note = CLP (coactosin-like protein)
NLVRDDGSAV

SEQ ID NO: 464 - protein, 9 aa, Homo sapiens
  PEPTIDE 1..9: note = CLP (coactosin-like protein)
RLFAFVRFT

SEQ ID NO: 465 - protein, 10 aa, Homo sapiens
  PEPTIDE 1..10: note = CLP (coactosin-like protein)
VVQNFAKEFV

SEQ ID NO: 466 - protein, 9 aa, Homo sapiens
  PEPTIDE 1..9: note = c-MET
YVDPVITSI

SEQ ID NO: 467 - protein, 9 aa, Homo sapiens
  PEPTIDE 1..9: note = CYP1B1
WLQYFPNPV

SEQ ID NO: 468 - protein, 9 aa, Homo sapiens
  PEPTIDE 1..9: note = IMP-3
NLSSAEVVV

SEQ ID NO: 469 - protein, 9 aa, Homo sapiens
  PEPTIDE 1..9: note = IMP-3
RLLVPTQFV

SEQ ID NO: 470 - protein, 9 aa, Homo sapiens
  PEPTIDE 1..9: note = KIF20A
LLSDDDVVV

SEQ ID NO: 471 - protein, 9 aa, Homo sapiens
  PEPTIDE 1..9: note = KIF20A
CIAEQYHTV

SEQ ID NO: 472 - protein, 10 aa, Homo sapiens
  PEPTIDE 1..10: note = KIF20A
AQPDTAPLPV

SEQ ID NO: 473 - protein, 9 aa, Homo sapiens
  PEPTIDE 1..9: note = MAGE-A10
SLLKFLAKV

SEQ ID NO: 474 - protein, 9 aa, Homo sapiens
  PEPTIDE 1..9: note = MAGE-A12
FLWGPRALV

SEQ ID NO: 475 - protein, 9 aa, Homo sapiens
  PEPTIDE 1..9: note = MAGE-C2
FLAKLNNTV

SEQ ID NO: 476 - protein, 9 aa, Homo sapiens
  PEPTIDE 1..9: note = Melan-A / MART-1
AAGIGILTV

SEQ ID NO: 477 - protein, 9 aa, Homo sapiens
  PEPTIDE 1..9: note = Survivin
QMFFCFKEL

SEQ ID NO: 478 - protein, 9 aa, Homo sapiens
  PEPTIDE 1..9: note = Telomerase
LLTSRLRFI

SEQ ID NO: 479 - protein, 10 aa, Homo sapiens
  PEPTIDE 1..10: note = TYMS
LMALPPCHAL

SEQ ID NO: 480 - protein, 9 aa, Homo sapiens
  PEPTIDE 1..9: note = cyclin D1
LLGATCMFV

SEQ ID NO: 481 - protein, 9 aa, Homo sapiens
  PEPTIDE 1..9: note = BAP31
KLDVGNAEV

SEQ ID NO: 482 - protein, 16 aa, Homo sapiens
  PEPTIDE 1..16: note = human MAGE3 243-258
KKLLTQHFVQENYLEY

SEQ ID NO: 483 - protein, 13 aa, Homo sapiens
  PEPTIDE 1..13: note = human oxytocinase 272-284
KKYFAATQFEPLA

SEQ ID NO: 484 - protein, 15 aa, Homo sapiens
  PEPTIDE 1..15: note = human CLIP 87-101
PVSKMRMATPLLMQA

SEQ ID NO: 485 - protein, 14 aa, Homo sapiens
  PEPTIDE 1..14: note = human CTAG1 157-170
SLLMWITQCFLPVF

SEQ ID NO: 486 - protein, 15 aa, Homo sapiens
  PEPTIDE 1..15: note = DQB1*03:02 human CLIP 87-101
PVSKMRMATPLLMQA

SEQ ID NO: 487 - protein, 16 aa, Homo sapiens
  PEPTIDE 1..16: note = human FcR2 104-119
QDLELSWNLNGLQADL

SEQ ID NO: 488 - protein, 9 aa, Homo sapiens
  PEPTIDE 1..9: note = Cancer-gp100
ALLAVGATK

SEQ ID NO: 489 - protein, 9 aa, synthetic construct
  PEPTIDE 1..9: note = HCMV pp65
GPISGHVLK

SEQ ID NO: 490 - protein, 10 aa, synthetic construct
  PEPTIDE 1..10: note = HCMV 248-256
AYAQKIFKIL

SEQ ID NO: 491 - protein, 10 aa, synthetic construct
  PEPTIDE 1..10: note = EBV-EBNA4
AVFDRKSDAK

SEQ ID NO: 492 - protein, 9 aa, synthetic construct
  PEPTIDE 1..9: note = EBV LMP2 CLG
CLGGLLTMV

SEQ ID NO: 493 - protein, 9 aa, synthetic construct
  PEPTIDE 1..9: note = EBV BMF1 GLC
GLCTLVAML

SEQ ID NO: 494 - protein, 9 aa, synthetic construct
  PEPTIDE 1..9: note = EBV LMP2 FLY
FLYALALLL

SEQ ID NO: 495 - protein, 9 aa, synthetic construct
  PEPTIDE 1..9: note = EBV BRLF1 YVL
YVLDHLIVV

SEQ ID NO: 496 - protein, 9 aa, synthetic construct
  PEPTIDE 1..9: note = EBV LMP2
IYVLVMLVL

SEQ ID NO: 497 - protein, 9 aa, synthetic construct
  PEPTIDE 1..9: note = EBV BRLF1
TYPVLEEMF

SEQ ID NO: 498 - protein, 9 aa, synthetic construct
  PEPTIDE 1..9: note = EBV BMLF1
DYNFVKQLF

SEQ ID NO: 499 - protein, 9 aa, synthetic construct
  PEPTIDE 1..9: note = EBV EBNA 3a RLR
RLRAEAQVK

SEQ ID NO: 500 - protein, 9 aa, synthetic construct
  PEPTIDE 1..9: note = EBV BRLF1 148-56 RVR
RVRAYTYSK

SEQ ID NO: 501 - protein, 9 aa, synthetic construct
  PEPTIDE 1..9: note = EBV EBNA RPP
RPPIFIRLL

SEQ ID NO: 502 - protein, 9 aa, synthetic construct
  PEPTIDE 1..9: note = EBV LMP2 FLY
FLYALALLL

SEQ ID NO: 503 - protein, 10 aa, synthetic construct
  PEPTIDE 1..10: note = EBV-E3B
LLDFVRFMGV

SEQ ID NO: 504 - protein, 9 aa, synthetic construct
  PEPTIDE 1..9: note = EBV-BALF4
FLDKGTYTL

SEQ ID NO: 505 - protein, 9 aa, synthetic construct
  PEPTIDE 1..9: note = EBV-BMRF1
TLDYKPLSV

SEQ ID NO: 506 - protein, 9 aa, synthetic construct
  PEPTIDE 1..9: note = EBV-LMP1
YLLEMLWRL

SEQ ID NO: 507 - protein, 9 aa, synthetic construct
  PEPTIDE 1..9: note = EBV-LMP1
YLQQNWWTL

SEQ ID NO: 508 - protein, 9 aa, synthetic construct
  PEPTIDE 1..9: note = Peptide
ILKEPVHGV

SEQ ID NO: 509 - protein, 10 aa, synthetic construct
  PEPTIDE 1..10: note = HIV pol
TPRVTGGGAM

SEQ ID NO: 510 - protein, 15 aa, synthetic construct
  PEPTIDE 1..15: note = HIV env 31-45
TEKLWVTVYYGVPVW

SEQ ID NO: 511 - protein, 9 aa, synthetic construct
  PEPTIDE 1..9: note = HIV-gag
SLYNTVATL

SEQ ID NO: 512 - protein, 8 aa, synthetic construct
  PEPTIDE 1..8: note = HIV
FLGKIWPS

SEQ ID NO: 513 - protein, 9 aa, synthetic construct
  PEPTIDE 1..9: note = Dextramer 1
GILGFVFTL

SEQ ID NO: 514 - protein, 9 aa, synthetic construct
  PEPTIDE 1..9: note = FLU BP-VSD
VSDGGPNLY

SEQ ID NO: 515 - protein, 9 aa, synthetic construct
  PEPTIDE 1..9: note = FLU NP 265-273 ILR
ILRGSVAHK

SEQ ID NO: 516 - protein, 10 aa, synthetic construct
  PEPTIDE 1..10: note = FLU-BNP
KLGEFYNQMM

SEQ ID NO: 517 - protein, 9 aa, synthetic construct
  PEPTIDE 1..9: note = VP1
DLQGLVLDY

SEQ ID NO: 518 - protein, 9 aa, synthetic construct
  PEPTIDE 1..9: note = VP1
VLGRKMTPK

SEQ ID NO: 519 - protein, 9 aa, synthetic construct
  PEPTIDE 1..9: note = VP1
VTLRKRWVK

SEQ ID NO: 520 - protein, 9 aa, synthetic construct
  PEPTIDE 1..9: note = VP1
LVLDYQTEY

SEQ ID NO: 521 - protein, 9 aa, synthetic construct
  PEPTIDE 1..9: note = VP1
GQEKTVYPK

SEQ ID NO: 522 - protein, 10 aa, synthetic construct
  PEPTIDE 1..10: note = VP1
VTFQSNQQDK

SEQ ID NO: 523 - protein, 10 aa, synthetic construct
  PEPTIDE 1..10: note = VP1
LKGPQKASQK

SEQ ID NO: 524 - protein, 11 aa, synthetic construct
  PEPTIDE 1..11: note = VP1
NVASVPKLLVK

SEQ ID NO: 525 - protein, 9 aa, synthetic construct
  PEPTIDE 1..9: note = VP1
TSNWYTYTY

SEQ ID NO: 526 - protein, 11 aa, synthetic construct
  PEPTIDE 1..11: note = VP1
LVLDYQTEYPK

SEQ ID NO: 527 - protein, 11 aa, synthetic construct
  PEPTIDE 1..11: note = VP1
TLRKRWVKNPY

SEQ ID NO: 528 - protein, 11 aa, synthetic construct
  PEPTIDE 1..11: note = VP1
AVTFQSNQQDK

SEQ ID NO: 529 - protein, 11 aa, synthetic construct
  PEPTIDE 1..11: note = VP1
PLKGPQKASQK

SEQ ID NO: 530 - protein, 9 aa, synthetic construct
  PEPTIDE 1..9: note = VP1
RIYEGSEQL

SEQ ID NO: 531 - protein, 9 aa, synthetic construct
  PEPTIDE 1..9: note = VP1
SLFSNLMPK

SEQ ID NO: 532 - protein, 10 aa, synthetic construct
  PEPTIDE 1..10: note = VP1
KLLVKGGVEV

SEQ ID NO: 533 - protein, 11 aa, synthetic construct
  PEPTIDE 1..11: note = VP1
SLINVHYWDMK

SEQ ID NO: 534 - protein, 10 aa, synthetic construct
  PEPTIDE 1..10: note = HPV E6 29-38
TIHDIILECV

SEQ ID NO: 535 - protein, 10 aa, synthetic construct
  PEPTIDE 1..10: note = HPV E7 11-20
YMLDLQPETT

SEQ ID NO: 536 - protein, 9 aa, synthetic construct
  PEPTIDE 1..9: note = VP1
GCCPNVASV

SEQ ID NO: 537 - protein, 9 aa, synthetic construct
  PEPTIDE 1..9: note = VP1
SITQIELYL

SEQ ID NO: 538 - protein, 9 aa, synthetic construct
  PEPTIDE 1..9: note = VP1
LQMWEAISV

SEQ ID NO: 539 - protein, 9 aa, synthetic construct
  PEPTIDE 1..9: note = VP1
AISVKTEVV

SEQ ID NO: 540 - protein, 9 aa, synthetic construct
  PEPTIDE 1..9: note = VP1
KMTPKNQGL

SEQ ID NO: 541 - protein, 9 aa, synthetic construct
  PEPTIDE 1..9: note = VP1
TVLQFSNTL

SEQ ID NO: 542 - protein, 9 aa, synthetic construct
  PEPTIDE 1..9: note = VP1
GLFISCADI

SEQ ID NO: 543 - protein, 10 aa, synthetic construct
  PEPTIDE 1..10: note = VP1
LLVKGGVEVL

SEQ ID NO: 544 - protein, 10 aa, synthetic construct
  PEPTIDE 1..10: note = VP1
ELYLNPRMGV

SEQ ID NO: 545 - protein, 10 aa, synthetic construct
  PEPTIDE 1..10: note = VP1
NLPAYSVARV

SEQ ID NO: 546 - protein, 10 aa, synthetic construct
  PEPTIDE 1..10: note = VP1
TLQMWEAISV

SEQ ID NO: 547 - protein, 10 aa, synthetic construct
  PEPTIDE 1..10: note = VP1
QMWEAISVKT

SEQ ID NO: 548 - protein, 10 aa, synthetic construct
  PEPTIDE 1..10: note = VP1
VVGISSLINV

SEQ ID NO: 549 - protein, 10 aa, synthetic construct
  PEPTIDE 1..10: note = VP1
SLINVHYWDM

SEQ ID NO: 550 - protein, 10 aa, synthetic construct
  PEPTIDE 1..10: note = VP1
HMFAIGGEPL

SEQ ID NO: 551 - protein, 10 aa, synthetic construct
  PEPTIDE 1..10: note = VP1
FAIGGEPLDL

SEQ ID NO: 552 - protein, 10 aa, synthetic construct
  PEPTIDE 1..10: note = VP1
NLINSLFSNL

SEQ ID NO: 553 - protein, 11 aa, synthetic construct
  PEPTIDE 1..11: note = VP1
FLFKTSGKMAL

SEQ ID NO: 554 - protein, 11 aa, synthetic construct
  PEPTIDE 1..11: note = VP1
ALHGLPRYFNV

SEQ ID NO: 555 - protein, 11 aa, synthetic construct
  PEPTIDE 1..11: note = VP1
NLINSLFSNLM

SEQ ID NO: 556 - protein, 11 aa, synthetic construct
  PEPTIDE 1..11: note = VP1
FLDKFGQEKTV

SEQ ID NO: 557 - protein, 10 aa, synthetic construct
  PEPTIDE 1..10: note = VP1
VKGGVEVLSV

SEQ ID NO: 558 - protein, 9 aa, synthetic construct
  PEPTIDE 1..9: note = VP1
ASVPKLLVK

SEQ ID NO: 559 - protein, 10 aa, synthetic construct
  PEPTIDE 1..10: note = VP1
CCPNVASVPK

SEQ ID NO: 560 - protein, 9 aa, synthetic construct
  PEPTIDE 1..9: note = VP1
ITIETVLGR

SEQ ID NO: 561 - protein, 9 aa, synthetic construct
  PEPTIDE 1..9: note = VP1
NTLTTVLLD

SEQ ID NO: 562 - protein, 9 aa, synthetic construct
  PEPTIDE 1..9: note = VP1
ALHGLPRYF

SEQ ID NO: 563 - protein, 10 aa, synthetic construct
  PEPTIDE 1..10: note = VP1
VASVPKLLVK

SEQ ID NO: 564 - protein, 9 aa, synthetic construct
  PEPTIDE 1..9: note = VP1
VSGQPMEGK

SEQ ID NO: 565 - protein, 10 aa, synthetic construct
  PEPTIDE 1..10: note = VP1
KASSTCKTPK

SEQ ID NO: 566 - protein, 10 aa, synthetic construct
  PEPTIDE 1..10: note = VP1
KTPKRQCIPK

SEQ ID NO: 567 - protein, 10 aa, synthetic construct
  PEPTIDE 1..10: note = VP1
YTYTYDLQPK

SEQ ID NO: 568 - protein, 10 aa, synthetic construct
  PEPTIDE 1..10: note = VP1
PITIETVLGR

SEQ ID NO: 569 - protein, 9 aa, synthetic construct
  PEPTIDE 1..9: note = VP1
SVARVSLPM

SEQ ID NO: 570 - protein, 10 aa, synthetic construct
  PEPTIDE 1..10: note = VP1
NSLFSNLMPK

SEQ ID NO: 571 - protein, 10 aa, synthetic construct
  PEPTIDE 1..10: note = VP1
KVSGQPMEGK

SEQ ID NO: 572 - protein, 10 aa, synthetic construct
  PEPTIDE 1..10: note = VP1
TVYPKPSVAP

SEQ ID NO: 573 - protein, 9 aa, synthetic construct
  PEPTIDE 1..9: note = VP1
GVEVLSVVT

SEQ ID NO: 574 - protein, 9 aa, synthetic construct
  PEPTIDE 1..9: note = VP1
PLDLQGLVL

SEQ ID NO: 575 - protein, 9 aa, synthetic construct
  PEPTIDE 1..9: note = VP1
GLDPQAKAK

SEQ ID NO: 576 - protein, 9 aa, synthetic construct
  PEPTIDE 1..9: note = VP1
EVWCPDPSK

SEQ ID NO: 577 - protein, 9 aa, synthetic construct
  PEPTIDE 1..9: note = VP1
ADIVGFLFK

SEQ ID NO: 578 - protein, 9 aa, synthetic construct
  PEPTIDE 1..9: note = VP1
KTSGKMALH

SEQ ID NO: 579 - protein, 9 aa, synthetic construct
  PEPTIDE 1..9: note = VP1
KMALHGLPR

SEQ ID NO: 580 - protein, 9 aa, synthetic construct
  PEPTIDE 1..9: note = VP1
RYFNVTLRK

SEQ ID NO: 581 - protein, 9 aa, synthetic construct
  PEPTIDE 1..9: note = VP1
TLRKRWVKN

SEQ ID NO: 582 - protein, 9 aa, synthetic construct
  PEPTIDE 1..9: note = VP1
KPGCCPNVA

SEQ ID NO: 583 - protein, 9 aa, synthetic construct
  PEPTIDE 1..9: note = VP1
QPIKENLPA

SEQ ID NO: 584 - protein, 9 aa, synthetic construct
  PEPTIDE 1..9: note = VP1
LPRYFNVTL

SEQ ID NO: 585 - protein, 9 aa, synthetic construct
  PEPTIDE 1..9: note = VP1
MPKVSGQPM

SEQ ID NO: 586 - protein, 9 aa, synthetic construct
  PEPTIDE 1..9: note = VP1
YPKPSVAPA

SEQ ID NO: 587 - protein, 9 aa, synthetic construct
  PEPTIDE 1..9: note = VP1
KPSVAPAAV

SEQ ID NO: 588 - protein, 9 aa, synthetic construct
  PEPTIDE 1..9: note = VP1
APLKGPQKA

SEQ ID NO: 589 - protein, 10 aa, synthetic construct
  PEPTIDE 1..10: note = VP1
APKRKASSTC

SEQ ID NO: 590 - protein, 10 aa, synthetic construct
  PEPTIDE 1..10: note = VP1
SVARVSLPML

SEQ ID NO: 591 - protein, 10 aa, synthetic construct
  PEPTIDE 1..10: note = VP1
YPKTTNGGPI

SEQ ID NO: 592 - protein, 10 aa, synthetic construct
  PEPTIDE 1..10: note = VP1
YPKPSVAPAA

SEQ ID NO: 593 - protein, 11 aa, synthetic construct
  PEPTIDE 1..11: note = VP1
KPGCCPNVASV

SEQ ID NO: 594 - protein, 11 aa, synthetic construct
  PEPTIDE 1..11: note = VP1
NPRMGVNSPDL

SEQ ID NO: 595 - protein, 11 aa, synthetic construct
  PEPTIDE 1..11: note = VP1
LPAYSVARVSL

SEQ ID NO: 596 - protein, 11 aa, synthetic construct
  PEPTIDE 1..11: note = VP1
TPTVLQFSNTL

SEQ ID NO: 597 - protein, 11 aa, synthetic construct
  PEPTIDE 1..11: note = VP1
LPRYFNVTLRK

SEQ ID NO: 598 - protein, 11 aa, synthetic construct
  PEPTIDE 1..11: note = VP1
YPVVNLINSLF

SEQ ID NO: 599 - protein, 11 aa, synthetic construct
  PEPTIDE 1..11: note = VP1
YPKPSVAPAAV

SEQ ID NO: 600 - protein, 11 aa, synthetic construct
  PEPTIDE 1..11: note = VP1
KPSVAPAAVTF

SEQ ID NO: 601 - protein, 9 aa, synthetic construct
  PEPTIDE 1..9: note = VP1
APKRKASST

SEQ ID NO: 602 - protein, 9 aa, synthetic construct
  PEPTIDE 1..9: note = HSV-1gB
RMLGDVMAV

SEQ ID NO: 603 - protein, 9 aa, synthetic construct
  PEPTIDE 1..9: note = HSV1gB
GIFEDRAPV

SEQ ID NO: 604 - protein, 9 aa, synthetic construct
  PEPTIDE 1..9: note = HSV1gB
YLANGGFLI

SEQ ID NO: 605 - protein, 10 aa, synthetic construct
  PEPTIDE 1..10: note = HPV-E7
LLMGTLGIVC

SEQ ID NO: 606 - protein, 9 aa, synthetic construct
  PEPTIDE 1..9: note = HSV-Ul25
FLWEDQTLL